European Patent Application EP 4 678 180 A1, published January 14, 2026. Title: A pharmaceutical composition for preventing or treating cancer comprising IL-2 analog or conjugate thereof. Applicant: HANMI PHARM. CO., LTD. Application KR. The sequence listing filed with the application follows.

SEQUENCE LISTING (439 sequences)

SEQ ID NO: 1 - protein, 133 aa, homo sapiens [sequence omitted]

SEQ ID NO: 2 - protein, 132 aa, synthetic construct
  REGION 1..132: note = IL-2 analog 1
PTSSSTKKTQLQLEHLLLDLQMILNGINNYKNPKLTRMLTFKFYMPKKATELKHLQCLEEELKPLEEVLNLAQSKNFHLRPRDLISNINVIVLELKGSETTFMCEYADETATIVEFLNRWITFSQSIISTLT

SEQ ID NO: 3 - protein, 132 aa, synthetic construct
  REGION 1..132: note = IL-2 analog 2
PTSSSTKKTQLQLEHLLLDLQMILNGINNYKNPKLTRMLTFKFYMPKKATELKHLQCLEEELKPLEEVLNLAQSKNFHLRPRDLICNINVIVLELKGSETTFMCEYADETATIVEFLNRWITFSQSIISTLT

SEQ ID NO: 4 - protein, 132 aa, synthetic construct
  REGION 1..132: note = IL-2 analog 3
PTSSSTKKTQLQLEHLLLDLQMILNGINNYCNPKLTRMLTFKFYMPKKATELKHLQCLEEELKPLEEVLNLAQSKNFHLRPRDLISNINVIVLELKGSETTFMCEYADETATIVEFLNRWITFSQSIISTLT

SEQ ID NO: 5 - protein, 132 aa, synthetic construct
  REGION 1..132: note = IL-2 analog 4
PTSSSTKKTQLQLEHLLLDLQMILNGINNYKNPCLTRMLTFKFYMPKKATELKHLQCLEEELKPLEEVLNLAQSKNFHLRPRDLISNINVIVLELKGSETTFMCEYADETATIVEFLNRWITFSQSIISTLT

SEQ ID NO: 6 - protein, 132 aa, synthetic construct
  REGION 1..132: note = IL-2 analog 5
PTSSSTKKTQLQLEHLLLDLQMILNGINNYKNPKLTRMLTFCFYMPKKATELKHLQCLEEELKPLEEVLNLAQSKNFHLRPRDLISNINVIVLELKGSETTFMCEYADETATIVEFLNRWITFSQSIISTLT

SEQ ID NO: 7 - protein, 132 aa, synthetic construct
  REGION 1..132: note = IL-2 analog 6
PTSSSTKKTQLQLEHLLLDLQMILNGINNYKNPKLTRMLTFKFYMPCKATELKHLQCLEEELKPLEEVLNLAQSKNFHLRPRDLISNINVIVLELKGSETTFMCEYADETATIVEFLNRWITFSQSIISTLT

SEQ ID NO: 8 - protein, 132 aa, synthetic construct
  REGION 1..132: note = IL-2 analog 7
PTSSSTKKTQLQLEHLLLDLQMILNGINNYKNPKLTRMLTFKFYMPKCATELKHLQCLEEELKPLEEVLNLAQSKNFHLRPRDLISNINVIVLELKGSETTFMCEYADETATIVEFLNRWITFSQSIISTLT

SEQ ID NO: 9 - protein, 132 aa, synthetic construct
  REGION 1..132: note = IL-2 analog 9
PTSSSTKKTQLQLEHLLLDLQMILNGINNYKNPKLTRMLTFKFYMPKKATELKHLQCLEEELKPLEEVLNLAQSCNFHLRPRDLISNINVIVLELKGSETTFMCEYADETATIVEFLNRWITFSQSIISTLT

SEQ ID NO: 10 - protein, 132 aa, synthetic construct
  REGION 1..132: note = IL-2 analog 10
PTSSSTKKTQLQLEHLLLDLQMILNGINNYKNPKLTAMLTFKFYMPKKATELKHLQCLEEELKPLEEVLNLAQSKNFHLRPRDLISNINVIVLELKGSETTFMCEYADETATIVEFLNRWITFSQSIISTLT

SEQ ID NO: 11 - protein, 132 aa, synthetic construct
  REGION 1..132: note = IL-2 analog 10
PTSSSTKKTQLQLEHLLLDLQMILNGINNYKNPKLTRMLTKKFYMPKKATELKHLQCLEEELKPLEEVLNLAQSKNFHLRPRDLISNINVIVLELKGSETTFMCEYADETATIVEFLNRWITFSQSIISTLT

SEQ ID NO: 12 - protein, 132 aa, synthetic construct
  REGION 1..132: note = IL-2 analog 11
PTSSSTKKTQLQLEHLLLDLQMILNGINNYKNPKLTRMLTAKFYMPKKATELKHLQCLEEELKPLEEVLNLAQSKNFHLRPRDLISNINVIVLELKGSETTFMCEYADETATIVEFLNRWITFSQSIISTLT

SEQ ID NO: 13 - protein, 132 aa, synthetic construct
  REGION 1..132: note = IL-2 analog 12
PTSSSTKKTQLQLEHLLLDLQMILNGINNYKNPKLTAMLTKKFYMPKKATELKHLQCLEEELKPLEEVLNLAQSKNFHLRPRDLISNINVIVLELKGSETTFMCEYADETATIVEFLNRWITFSQSIISTLT

SEQ ID NO: 14 - protein, 132 aa, synthetic construct
  REGION 1..132: note = IL-2 analog 13
PTSSSTKKTQLQLEHLLLDLQMILNGINNYKNPKLTAMLTAKFYMPKKATELKHLQCLEEELKPLEEVLNLAQSKNFHLRPRDLISNINVIVLELKGSETTFMCEYADETATIVEFLNRWITFSQSIISTLT

SEQ ID NO: 15 - protein, 132 aa, synthetic construct
  REGION 1..132: note = IL-2 analog 14
PTSSSTKKTQLQLEHLLYDLQMILNGINNYKNPKLTAMLTKKFYMPKKATELKHLQCLEEELKPLEEVLNLAQSKNFHLRPRDLISNINVIVLELKGSETTFMCEYADETATIVEFLNRWITFSQSIISTLT

SEQ ID NO: 16 - protein, 132 aa, synthetic construct
  REGION 1..132: note = IL-2 analog 15
PTSSSTKKTQLQLEHLLLDLQMILNGINNYKNPKLTAMLTKKFYMPKKATELKHLQCLEEELKPLEEVLNLAQSKNFHLRPRELISNINVIVLELKGSETTFMCEYADETATIVEFLNRWITFSQSIISTLT

SEQ ID NO: 17 - protein, 132 aa, synthetic construct
  REGION 1..132: note = IL-2 analog 16
PTSSSTKKTQLQLEHLLLDLQMILNGINNYKNPKLTAMLTKKFYMPKKATELKHLQCLEEELKPLEEVLNLAQSKNFHLRPRDLISQINVIVLELKGSETTFMCEYADETATIVEFLNRWITFSQSIISTLT

SEQ ID NO: 18 - protein, 132 aa, synthetic construct
  REGION 1..132: note = IL-2 analog 17
PTSSSTKKTQLQLEHLLLDLQMILNGINNYKNPKLTAMLTKKFYMPKKATELKHLQCLEEELKPLEEVLNLAQSKNFHLRPRDLISNINTIVLELKGSETTFMCEYADETATIVEFLNRWITFSQSIISTLT

SEQ ID NO: 19 - protein, 132 aa, synthetic construct
  REGION 1..132: note = IL-2 analog 18
PTSSSTKKTQLQLEHLLLDLQMILNGINNYKNPKLTAMLTKKFYMPKKATELKHLQCLEQELKPLEEVLNLAQSKNFHLRPRDLISNINVIVLELKGSETTFMCEYADETATIVEFLNRWITFSQSIISTLT

SEQ ID NO: 20 - protein, 132 aa, synthetic construct
  REGION 1..132: note = IL-2 analog 19
PTSSSTKKTQLQLEHLLLDLQMILNGINNYKNPKLTAMLTKKFYMPKKATELKHLQCLEEELKPLEEVLNLAQSKNFHLDPRDLISNINVFVLELKGSETTFMCEYADETATIVEFLNRWITFSQSIISTLT

SEQ ID NO: 21 - protein, 132 aa, synthetic construct
  REGION 1..132: note = IL-2 analog 20
PTSSSTKKTQLQLEHLLLDLQMILNGINNYKNPKLTAMLTKKFYMPKKATELKHLQCLEEELKPLEEVLNLAQSKNFHLRPRDVVSNINVFVLELKGSETTFMCEYADETATIVEFLNRWITFSQSIISTLT

SEQ ID NO: 22 - protein, 132 aa, synthetic construct
  REGION 1..132: note = IL-2 analog 21
PTSSSTKKTQLQLEHLLLDLQMILNGINNYKNPKLTAMLTKKFYMPKKATELKHLQCLEEELKPLEEVLNLAQSKNFHFDPRDVVSNINVFVLELKGSETTFMCEYADETATIVEFLNRWITFSQSIISTLT

SEQ ID NO: 23 - protein, 132 aa, synthetic construct
  REGION 1..132: note = IL-2 analog 22
PTSSSTKKTQVQLEHLLLDLQMILNGINNYKNPKLTAMLTKKFYMPKKATELKHLQCLEEELKPLEEVLNLAQSKNFHLRPRDLISNINVIVLELKGSETTFMCEYADETATIVEFLNRWITFSQSIISTLT

SEQ ID NO: 24 - protein, 132 aa, synthetic construct
  REGION 1..132: note = IL-2 analog 23
PTSSSTKKTQFQLEHLLLDLQMILNGINNYKNPKLTAMLTKKFYMPKKATELKHLQCLEEELKPLEEVLNLAQSKNFHLRPRDLISNINVIVLELKGSETTFMCEYADETATIVEFLNRWITFSQSIISTLT

SEQ ID NO: 25 - protein, 132 aa, synthetic construct
  REGION 1..132: note = IL-2 analog 24
PTSSSTKKTQLQLEHLLVDLQMILNGINNYKNPKLTAMLTKKFYMPKKATELKHLQCLEEELKPLEEVLNLAQSKNFHLRPRDLISNINVIVLELKGSETTFMCEYADETATIVEFLNRWITFSQSIISTLT

SEQ ID NO: 26 - protein, 132 aa, synthetic construct
  REGION 1..132: note = IL-2 analog 25
PTSSSTKKTQLQLEHLLFDLQMILNGINNYKNPKLTAMLTKKFYMPKKATELKHLQCLEEELKPLEEVLNLAQSKNFHLRPRDLISNINVIVLELKGSETTFMCEYADETATIVEFLNRWITFSQSIISTLT

SEQ ID NO: 27 - protein, 132 aa, synthetic construct
  REGION 1..132: note = IL-2 analog 26
PTSSSTKKTQLQLEHLLLDLQMILNGINNYKNPKLTAMLTKKFYMPKKATELKHLQCLEEELKPLEEVLNLAQSKNFHLRPRDLISNFNVIVLELKGSETTFMCEYADETATIVEFLNRWITFSQSIISTLT

SEQ ID NO: 28 - protein, 132 aa, synthetic construct
  REGION 1..132: note = IL-2 analog 27
PTSSSTKKTQLQLEHLLLDLQMILNGINNYKNPKLTAMLTKKFYMPKKATELKHLQCLEEELKPLEEVLNLAQSKNFHLRPRDLISNINFIVLELKGSETTFMCEYADETATIVEFLNRWITFSQSIISTLT

SEQ ID NO: 29 - protein, 132 aa, synthetic construct
  REGION 1..132: note = IL-2 analog 28
PTSSSTKKTQLQLEHLLLDLQMILNGINNYKNPKLTAMLTKKFYMPKKATELKHLQCLEEELKPLEEVLNLAQSKNFHLRPRDLISNINVIVVELKGSETTFMCEYADETATIVEFLNRWITFSQSIISTLT

SEQ ID NO: 30 - protein, 132 aa, synthetic construct
  REGION 1..132: note = IL-2 analog 29
PTSSSTKKTQLQLEHLLLDLQMILNGINNYKNPKLTAMLTKKFYMPKKATELKHLQCLEEELKPLEEVLNLAQSKNFHLRPRDLISNINVIVLELKGSETTFMCEYADETATIVEFLNRWITFSTSIISTLT

SEQ ID NO: 31 - protein, 132 aa, synthetic construct
  REGION 1..132: note = IL-2 analog 30
PTSSSTKKTQLQLEHLLLDLQMILNGINNYKNPKLTAMLTFKFYMPKKATELKHLQCLEEELKPLEEVLNLAQSKNFHLDPRDLISNINVFVLELKGSETTFMCEYADETATIVEFLNRWITFSQSIISTLT

SEQ ID NO: 32 - protein, 132 aa, synthetic construct
  REGION 1..132: note = IL-2 analog 31
PTSSSTKKTQLQLEHLLLDLQMILNGINNYKNPKLTAMLTFKFYMPKKATELKHLQCLEEELKPLEEVLNLAQSKNFHLRPRELISNINVIVLELKGSETTFMCEYADETATIVEFLNRWITFSQSIISTLT

SEQ ID NO: 33 - protein, 132 aa, synthetic construct
  REGION 1..132: note = IL-2 analog 32
PTSSSTKKTQLQLEHLLLDLQMILNGINNYKNPKLTAMLTFKFYMPKKATELKHLQCLEEELKPLEEVLNLAQSKNFHLDPRELISNINVFVLELKGSETTFMCEYADETATIVEFLNRWITFSQSIISTLT

SEQ ID NO: 34 - protein, 132 aa, synthetic construct
  REGION 1..132: note = IL-2 analog 33
PTSSSTKKTQLQLEHLLLDLQMILNGINNYKNPKLTAMLTFKFYMPKKATELKHLQCLEEELKPLEEVLNLAQSKNFHFRPRDLISNINVIVLELKGSETTFMCEYADETATIVEFLNRWITFSQSIISTLT

SEQ ID NO: 35 - protein, 132 aa, synthetic construct
  REGION 1..132: note = IL-2 analog 34
PTSSSTKKTQLQLEHLLLDLQMILNGINNYKNPKLTAMLTFKFYMPKKATELKHLQCLEEELKPLEEVLNLAQSKNFHFRPRELISNINVIVLELKGSETTFMCEYADETATIVEFLNRWITFSQSIISTLT

SEQ ID NO: 36 - protein, 132 aa, synthetic construct
  REGION 1..132: note = IL-2 analog 35
PTSSSTKKTQLQLEHLLLDLQMILNGINNYKNPKLTAMLTFKFYMPKKATELKHLQCLEEELKPLEEVLNLAQSKNFHLRPRDLISNINVIVFEFKGSETTFMCEYADETATIVEFLNRWITFSQSIISTLT

SEQ ID NO: 37 - protein, 132 aa, synthetic construct
  REGION 1..132: note = IL-2 analog 36
PTSSSTKKTQLQLEHLLLDLQMILNGINNYKNPKLTAMLTFKFYMPKKATELKHLQCLEEELKPLEEVLNLAQSKNFHLRPRDLISNINVIVFEVKGSETTFMCEYADETATIVEFLNRWITFSQSIISTLT

SEQ ID NO: 38 - protein, 132 aa, synthetic construct
  REGION 1..132: note = IL-2 analog 37
PTSSSTKKTQLQLEHLLLDLQMILNGINNYKNPKLTAMLTFKFYMPKKATELKHLQCLEEELKPLEEVLNLAQSKNFHLRPRDLISNINVIVFEIKGSETTFMCEYADETATIVEFLNRWITFSQSIISTLT

SEQ ID NO: 39 - protein, 132 aa, synthetic construct
  REGION 1..132: note = IL-2 analog 38
PTSSSTKKTQLQLEHLLLDLQMILNGINNYKNPKLTAMLTKKFYMPKKATELKHLQCLEEELKPLEEVLNLAQSKNFHLDPRDLISNINVFVFEFKGSETTFMCEYADETATIVEFLNRWITFSQSIISTLT

SEQ ID NO: 40 - protein, 132 aa, synthetic construct
  REGION 1..132: note = IL-2 analog 39
PTSSSTKKTQLQLEHLLLDLQMILNGINNYKNPKLTAMLTKKFYMPKKATELKHLQCLEEELKPLEEVLNLAQSKNFHLDPRDLISNINVFVFEVKGSETTFMCEYADETATIVEFLNRWITFSQSIISTLT

SEQ ID NO: 41 - protein, 132 aa, synthetic construct
  REGION 1..132: note = IL-2 analog 40
PTSSSTKKTQLQLEHLLLDLQMILNGINNYKNPKLTAMLTKKFYMPKKATELKHLQCLEEELKPLEEVLNLAQSKNFHLDPRDLISNINVFVFEIKGSETTFMCEYADETATIVEFLNRWITFSQSIISTLT

SEQ ID NO: 42 - protein, 132 aa, synthetic construct
  REGION 1..132: note = IL-2 analog 41
PTSSSTKKTQLQLEHLLLDLQMILNGINNYKNPKLTRMLTFKFYMPKKATELKHLQCLEEELKPLEEVLNLAQSKNFHFDPRDVVSNINVFVLELKGSETTFMCEYADETATIVEFLNRWITFSQSIISTLT

SEQ ID NO: 43 - protein, 132 aa, synthetic construct
  REGION 1..132: note = IL-2 analog 42
PTSSSTKKTQLQLEHLLLDLQMILNGINNYKNPKLTAMLTKKFYMPKKATELKHLQCLEEELKPLEEVLNLAQSKNFHLEPRDLISNINVFVLELKGSETTFMCEYADETATIVEFLNRWITFSQSIISTLT

SEQ ID NO: 44 - protein, 132 aa, synthetic construct
  REGION 1..132: note = IL-2 analog 43
PTSSSTKKTQLQLEHLLLDLQMILNGINNYKNPKLTAMLTKKFYMPKKATELKHLQCLEEELKPLEEVLNLAQSKNFHLDPRDLISNINVLVLELKGSETTFMCEYADETATIVEFLNRWITFSQSIISTLT

SEQ ID NO: 45 - protein, 132 aa, synthetic construct
  REGION 1..132: note = IL-2 analog 44
PTSSSTKKTQLQLEHLLLDLQMILNGINNYKNPKLTAMLTKKFYMPKKATELKHLQCLEEELKPLEEVLNLAQSKNFHLDPRVLISNINVFVLELKGSETTFMCEYADETATIVEFLNRWITFSQSIISTLT

SEQ ID NO: 46 - protein, 132 aa, synthetic construct
  REGION 1..132: note = IL-2 analog 45
PTSSSTKKTQLQLEHLLLDLQMILNGINNYKNPKLTAMLTKKFYMPKKATELKHLQCLEEELKPLEEVLNLAQSKNFHLDPRFLISNINVFVLELKGSETTFMCEYADETATIVEFLNRWITFSQSIISTLT

SEQ ID NO: 47 - protein, 132 aa, synthetic construct
  REGION 1..132: note = IL-2 analog 46
PTSSSTKKTQLQLEHLLLVLQMILNGINNYKNPKLTAMLTKKFYMPKKATELKHLQCLEEELKPLEEVLNLAQSKNFHLDPRDLISNINVFVLELKGSETTFMCEYADETATIVEFLNRWITFSQSIISTLT

SEQ ID NO: 48 - protein, 132 aa, synthetic construct
  REGION 1..132: note = IL-2 analog 47
PTSSSTKKTQLQLEHLLLFLQMILNGINNYKNPKLTAMLTKKFYMPKKATELKHLQCLEEELKPLEEVLNLAQSKNFHLDPRDLISNINVFVLELKGSETTFMCEYADETATIVEFLNRWITFSQSIISTLT

SEQ ID NO: 49 - protein, 132 aa, synthetic construct
  REGION 1..132: note = IL-2 analog 48
PTSSSTKKTQLQLEHLLLDLQMILNGINNYKNPKLTAMLTKKFYMPKKATELKHLQCLEEELKPLEEVLNLAQSKNFHLDPRDLISVINVFVLELKGSETTFMCEYADETATIVEFLNRWITFSQSIISTLT

SEQ ID NO: 50 - protein, 132 aa, synthetic construct
  REGION 1..132: note = IL-2 analog 49
PTSSSTKKTQLQLEHLLLDLQMILNGINNYKNPKLTAMLTKKFYMPKKATELKHLQCLEEELKPLEEVLNLAQSKNFHLDPRDLISFINVFVLELKGSETTFMCEYADETATIVEFLNRWITFSQSIISTLT

SEQ ID NO: 51 - protein, 132 aa, synthetic construct
  REGION 1..132: note = IL-2 analog 50
PTSSSTKKTQLQLEHLLLDLQMILNGINNYKNPKLTRMLTKKFYMPKKATELKHLQCLEEELKPLEEVLNLAQSKNFHFDPRDVVSNINVFVLELKGSETTFMCEYADETATIVEFLNRWITFSQSIISTLT

SEQ ID NO: 52 - protein, 132 aa, synthetic construct
  REGION 1..132: note = IL-2 analog 51
PTSSSTKKTQLQLEHLLLDLQMILNGINNYKNPKLTRMLTFKFYMPKKATELKHLQCLEQELKPLEEVLNLAQSKNFHLDPRDLISNINVFVLELKGSETTFMCEYADETATIVEFLNRWITFSQSIISTLT

SEQ ID NO: 53 - protein, 132 aa, synthetic construct
  REGION 1..132: note = IL-2 analog 52
PTSSSTKKTQLQLEHLLLDLQMILNGINNYKNPKLTAMLTKKFYMPKKATELKHLQCLEEELKPLEEVLNLAQSKNFHFDPRDLISNINVFVLELKGSETTFMCEYADETATIVEFLNRWITFSQSIISTLT

SEQ ID NO: 54 - protein, 132 aa, synthetic construct
  REGION 1..132: note = IL-2 analog 53
PTSSSTKKTQLQLEHLLLDLQMILNGINNYKNPKLTAMLTKKFYMPKKATELKHLQCLEEELKPLEEVLNLAQSKNFHFDPRELISNINVFVLELKGSETTFMCEYADETATIVEFLNRWITFSQSIISTLT

SEQ ID NO: 55 - protein, 132 aa, synthetic construct
  REGION 1..132: note = IL-2 analog 54
PTSSSTKKTQLQLEHLLLDLQMILNGINNYKNPKLTAMLTKKFYMPKKATELKHLQCLEEELKPLEEVLNLAHSKNFHLDPRDLISNINVFVLELKGSETTFMCEYADETATIVEFLNRWITFSQSIISTLT

SEQ ID NO: 56 - protein, 132 aa, synthetic construct
  REGION 1..132: note = IL-2 analog 55
PTSSSTKKTQLQLEHLLLDLQMILNGINNYKNPKLTAMLTKKFYMPKKATELKHLQCLEEELKPLEEVLNLAHSKNFHFDPRDLISNINVFVLELKGSETTFMCEYADETATIVEFLNRWITFSQSIISTLT

SEQ ID NO: 57 - protein, 132 aa, synthetic construct
  REGION 1..132: note = IL-2 analog 56
PTSSSTKKTQLQLEHLLLDLQMILNGINNYKNPKLTAMLTKKFAMPKKATELKHLQCLEEELKPLEEVLNLAHSKNFHLDPRDLISNINVFVLELKGSETTFMCEYADETATIVEFLNRWITFSQSIISTLT

SEQ ID NO: 58 - protein, 132 aa, synthetic construct
  REGION 1..132: note = IL-2 analog 57
PTSSSTKKTQLQLEHLLLDLQMILNGINNYKNPKLTAMLTKKFAMPKKATELKHLQCLEEELKPLEEVLNLAHSKNFHFDPRDLISNINVFVLELKGSETTFMCEYADETATIVEFLNRWITFSQSIISTLT

SEQ ID NO: 59 - protein, 132 aa, synthetic construct
  REGION 1..132: note = IL-2 analog 61
PTSSSTKKTQLQLEHLLLDLQMILNGINNYKNPKLTAMLTKKFYMPKKATELKHLQCLEEELKPLEEVLNLAQSKNFHFDPRDAASNINVYVLELKGSETTFMCEYADETATIVEFLNRWITFSQSIISTLT

SEQ ID NO: 60 - protein, 132 aa, synthetic construct; identical to SEQ ID NO: 59
  REGION 1..132: note = IL-2 analog 59

SEQ ID NO: 61 - protein, 132 aa, synthetic construct
  REGION 1..132: note = IL-2 analog 60
PTSSSTKKTQLQLEHLLLDLQMILNGINNYKNPKLTAMLTKKFAMPKKATELKHLQCLEEELKPLEEVLNLAQSKNFHYRPRDAASNINVYVLELKGSETTFMCEYADETATIVEFLNRWITFSQSIISTLT

SEQ ID NO: 62 - protein, 132 aa, synthetic construct
  REGION 1..132: note = IL-2 analog 61
PTSSSTKKTQLQLEHLLLDLQMILNGINNYKNPKLTAMLTKKFYMPKKATELKHLQCLEEELKPLEEVLNLAQSKNFHYDPRDGVSNINVYVLELKGSETTFMCEYADETATIVEFLNRWITFSQSIISTLT

SEQ ID NO: 63 - protein, 132 aa, synthetic construct
  REGION 1..132: note = IL-2 analog 62
PTSSSTKKTQLQLEHLLLDLQMILNGINNYKNPKLTAMLTKKFYMPKKATELKHLQCLEEELKPLEEVLNLAQSKNFHWEPRDGASNINVFVLELKGSETTFMCEYADETATIVEFLNRWITFSQSIISTLT

SEQ ID NO: 64 - protein, 132 aa, synthetic construct
  REGION 1..132: note = IL-2 analog 63
PTSSSTKKTQLQLEHLLLDLQMILNGINNYKNPKLTAMLTKKFYMPKKATELKHLQCLEEELKPLEEVLNLAQSKNFHDEPRDTGSNINVFVLELKGSETTFMCEYADETATIVEFLNRWITFSQSIISTLT

SEQ ID NO: 65 - protein, 132 aa, synthetic construct
  REGION 1..132: note = IL-2 analog 64
PTSSSTKKTQLQLEHLLLDLQMILNGINNYKNPKLTAMLTKKFYMPKKATELKHLQCLEEELKPLEEVLNLAQSKNFHYNPRDVVSNINVYVLELKGSETTFMCEYADETATIVEFLNRWITFSQSIISTLT

SEQ ID NO: 66 - protein, 132 aa, synthetic construct
  REGION 1..132: note = IL-2 analog 65
PTSSSTKKTQLQLEHLLLDLQMILNGINNYKNPKLTAMLTKKFYMPKKATELKHLQCLEEELKPLEEVLNLAQSKNFHYEPRDVVSNINVFVLELKGSETTFMCEYADETATIVEFLNRWITFSQSIISTLT

SEQ ID NO: 67 - protein, 132 aa, synthetic construct
  REGION 1..132: note = IL-2 analog 66
PTSSSTKKTQLQLEHLLLDLQMILNGINNYKNPKLTAMLTKKFYMPKKATELKHLQCLEEELKPLEEVLNLAQSKNFHFEPRDFVSNINVFVLELKGSETTFMCEYADETATIVEFLNRWITFSQSIISTLT

SEQ ID NO: 68 - protein, 132 aa, synthetic construct
  REGION 1..132: note = IL-2 analog 67
PTSSSTKKTQLQLEHLLLDLQMILNGINNYKNPKLTAMLTKKFYMPKKATELKHLQCLEEELKPLEEVLNLAQSKNFHYDPRDFVSNINVWVLDLKGSETTFMCEYADETATIVEFLNRWITFSQSIISTLT

SEQ ID NO: 69 - protein, 132 aa, synthetic construct
  REGION 1..132: note = IL-2 analog 68
PTSSSTKKTQLQLEHLLLDLQMILNGINNYKNPKLTAMLTKKFYMPKKATELKHLQCLEEELKPLEEVLNLAQSKNFHFEPRDIVSNINEFVLELKGSETTFMCEYADETATIVEFLNRWITFSQSIISTLT

SEQ ID NO: 70 - protein, 132 aa, synthetic construct
  REGION 1..132: note = IL-2 analog 69
PTSSSTKKTQLQLEHLLLDLQMILNGINNYKNPKLTAMLTKKFYMPKKATELKHLQCLEEELKPLEEVLNLAQSKNFHYEPRDFLSNINEWVLDLKGSETTFMCEYADETATIVEFLNRWITFSQSIISTLT

SEQ ID NO: 71 - protein, 132 aa, synthetic construct
  REGION 1..132: note = IL-2 analog 70
PTSSSTKKTQLQLEHLLLDLQMILNGINNYKNPKLTAMLTKKFYMPKKATELKHLQCLEEELKPLEEVLNLAQSKNFHYDPRDVVSNINVFVLELKGSETTFMCEYADETATIVEFLNRWITFSQSIISTLT

SEQ ID NO: 72 - protein, 132 aa, synthetic construct
  REGION 1..132: note = IL-2 analog 71
PTSSSTKKTQLQLEHLLLDLQMILNGINNYKNPKLTAMLTKKFYMPKKATELKHLQCLEEELKPLEEVLNLAQSKNFHFEPRDVVSNINVFVLELKGSETTFMCEYADETATIVEFLNRWITFSQSIISTLT

SEQ ID NO: 73 - protein, 132 aa, synthetic construct
  REGION 1..132: note = IL-2 analog 72
PTSSSTKKTQLQLEHLLLDLQMILNGINNYKNPKLTAMLTKKFYMPKKATELKHLQCLEEELKPLEEVLNLAQSKNFHFDPRDVGSNINVFVLELKGSETTFMCEYADETATIVEFLNRWITFSQSIISTLT

SEQ ID NO: 74 - protein, 132 aa, synthetic construct
  REGION 1..132: note = IL-2 analog 73
PTSSSTKKTQLQLEHLLLDLQMILNGINNYKNPKLTAMLTKKFYMPKKATELKHLQCLEEELKPLEEVLNLAQSKNFHFDPRDWVSNINVFVLELKGSETTFMCEYADETATIVEFLNRWITFSQSIISTLT

SEQ ID NO: 75 - protein, 132 aa, synthetic construct
  REGION 1..132: note = IL-2 analog 74
PTSSSTKKTQLQLEHLLLDLQMILNGINNYKNPKLTDMLTKKFYMPKKATELKHLQCLEEELKPLEEVLNLAQSKNFHYDPRDVVSNINVFVLELKGSETTFMCEYADETATIVEFLNRWITFSQSIISTLT

SEQ ID NO: 76 - protein, 132 aa, synthetic construct
  REGION 1..132: note = IL-2 analog 75
PTSSSTKKTQLQLEHLLLDLQMILNGINNYKNPKLTAMLTKKFAMPKKATELKHLQCLEEELKPLEEVLNLAQSKNFHFEPRDVVSNINVFVLELKGSETTFMCEYADETATIVEFLNRWITFSQSIISTLT

SEQ ID NO: 77 - protein, 132 aa, synthetic construct
  REGION 1..132: note = IL-2 analog 76
PTSSSTKKTQLQLEHLLLDLQMILNGINNYKNPKLTAMLTKQFYMPKKATELKHLQCLERELKPLEEVLNLAQSKNFHFDPRDVGSNINVFVLELKGSETTFMCEYADETATIVEFLNRWITFSQSIISTLT

SEQ ID NO: 78 - protein, 132 aa, synthetic construct
  REGION 1..132: note = IL-2 analog 77
PTSSSTKKTQLQLEHLLLDLQMILNGINNYKNPKLTAMLTKEFYMPKKATELKHLQCLERELKPLEEVLNLAQSKNFHFDPRDWVSNINVFVLELKGSETTFMCEYADETATIVEFLNRWITFSQSIISTLT

SEQ ID NO: 79 - protein, 132 aa, synthetic construct
  REGION 1..132: note = IL-2 analog 78
PTSSSTKKTQLQLEHLLLDLQMILNGINNYKNPELTAMLTKKFYMPKKATELKHLQCLEEELKPLEEVLNLAQSKNFHFEPRDVVSNINVFVLELKGSETTFMCEYADETATIVEFLNRWITFSQSIISTLT

SEQ ID NO: 80 - protein, 132 aa, synthetic construct
  REGION 1..132: note = IL-2 analog 79
PTSSSTKKTQLQLEHLLLDLQMILNGINNYKNPELTAMLTKKFYMPKKATELKHLQCLEEELKPLEEVLNLAHSKNFHFEPRDVVSNINVFVLELKGSETTFMCEYADETATIVEFLNRWITFSQSIISTLT

SEQ ID NO: 81 - protein, 132 aa, synthetic construct
  REGION 1..132: note = IL-2 analog 80
PTSSSTKKTQLQLEHLLLDLQMILNGINNYKNPELTAMLTKKFYMPKKATELKHLQCLEEELKPLEEVLNLAHSKNFHFEGRDVVSNINVFVLELKGSETTFMCEYADETATIVEFLNRWITFSQSIISTLT

SEQ ID NO: 82 - protein, 132 aa, synthetic construct
  REGION 1..132: note = IL-2 analog 81
PTSSSTKKTQLQLEHLLLDLQMILNGINNYKNPELTAMLTKKFYMPKKATELKHLQCLEEELKPLEEVLNLAHSKNFHFEVRDVVSNINVFVLELKGSETTFMCEYADETATIVEFLNRWITFSQSIISTLT

SEQ ID NO: 83 - protein, 132 aa, synthetic construct
  REGION 1..132: note = IL-2 analog 82
PTSSSTKKTQLQLEHLRLDLEMILNGINNYKNPKLTRMLTFKFYMPKKATELKHLQCLEEELKPLEEVLNLAQSKNFHFDPRDEVSNINVFVLELKGSETTFMCEYADETATIVEFLNRWITFSQSIISTLT

SEQ ID NO: 84 - protein, 132 aa, synthetic construct
  REGION 1..132: note = IL-2 analog 83
PTSSSTKKTQLQLEHLRRDLEMILNGINNYKNPKLTRMLTFKFYMPKKATELKHLQCLEEELKPLEEVLNLAQSKNFHFDPRDEVSNINVFVLELKGSETTFMCEYADETATIVEFLNRWITFSQSIISTLT

SEQ ID NO: 85 - protein, 132 aa, synthetic construct
  REGION 1..132: note = IL-2 analog 84
PTSSSTKKTQLQLEHLRLDLEMILNGINNYKNPKLTRMLTFKFYMPKKATELKHLQCLEEELKPLEEVLNLAQSKNFHVDPRDEVSNINVFVLELKGSETTFMCEYADETATIVEFLNRWITFSQSIISTLT

SEQ ID NO: 86 - protein, 132 aa, synthetic construct
  REGION 1..132: note = IL-2 analog 85
PTSSSTKKTQLQLEHLLLDLQMILNGINNYKNPKLTRMLTFKFYMPKKATELKHLQCLEEELKPLEEVLNLAQSKNFHFEPRDVVSNINVFVLELKGSETTFMCEYADETATIVEFLNRWITFSQSIISTLT

SEQ ID NO: 87 - protein, 132 aa, synthetic construct
  REGION 1..132: note = IL-2 analog 86
PTSSSTKKTQLQLEHLRLDLEMILNGINNYKNPKLTRMLTFKFYMPKKATELKHLQCLEEELKPLEEVLNLAQSKNFHFEPRDVVSNINVFVLELKGSETTFMCEYADETATIVEFLNRWITFSQSIISTLT

SEQ ID NO: 88 - protein, 132 aa, synthetic construct
  REGION 1..132: note = IL-2 analog 87
PTSSSTKKTQLQLEHLRRDLEMILNGINNYKNPKLTRMLTFKFYMPKKATELKHLQCLEEELKPLEEVLNLAQSKNFHFEPRDVVSNINVFVLELKGSETTFMCEYADETATIVEFLNRWITFSQSIISTLT

SEQ ID NO: 89 - protein, 132 aa, synthetic construct
  REGION 1..132: note = IL-2 analog 88
PTSSSTKKTQLQLEHLLLDLQMILNGINNYKNPKLTRMLTFKFYMPKKATELKHLQCLEDELKPLEEVLNLAQSKNFHFEPRDVVSNINVFVLELKGSETTFMCEYADETATIVEFLNRWITFSQSIISTLT

SEQ ID NO: 90 - protein, 132 aa, synthetic construct
  REGION 1..132: note = IL-2 analog 89
PTSSSTKKTQLQLEHLLLDLQMILNGINNYKNPKLTAMLTFKFYMPKKATELKHLQCLEEELKPLEQVLNLAQSKNFHFEPRDVVSNINVFVLELKGSETTFMCEYADETATIVEFLNRWITFSQSIISTLT

SEQ ID NO: 91 - protein, 132 aa, synthetic construct
  REGION 1..132: note = IL-2 analog 90
PTSSSTKKTQLQLEHLLLDLQMILNGINNYKNPKLTRMLTWKFYMPKKATELKHLQCLEEELKPLEEVLNLAQSKNFHFEPRDVVSNINVFVLELKGSETTFMCEYADETATIVEFLNRWITFSQSIISTLT

SEQ ID NO: 92 - protein, 132 aa, synthetic construct
  REGION 1..132: note = IL-2 analog 91
PTSSSTKKTQLQLEHLLLDLQMILNGINNYKNPKLTRMLTFKFYMPKKATELKHLQCLEQELKPLEEVLNLAQSKNFHFEPRDVVSNINVFVLELKGSETTFMCEYADETATIVEFLNRWITFSQSIISTLT

SEQ ID NO: 93 - protein, 132 aa, synthetic construct
  REGION 1..132: note = IL-2 analog 92
PTSSSTKKTQLQLEHLLLDLQMILNGINNYKNPKLTRMLTFKFYMPKKATELKHLQCLEEELKPLEEVLNLAQSKNFHFEPRDVVSNINTFVLELKGSETTFMCEYADETATIVEFLNRWITFSQSIISTLT

SEQ ID NO: 94 - protein, 132 aa, synthetic construct
  REGION 1..132: note = IL-2 analog 93
PTSSSTKKTQLQLEHLLLDLQMILNGINNYKNPKLTRMLTFKFYMPKKATELKHLQCLEEELKPLEEVLNLAQSKNFHFEPREVVSNINTFVLELKGSETTFMCEYADETATIVEFLNRWITFSQSIISTLT

SEQ ID NO: 95 - protein, 132 aa, synthetic construct
  REGION 1..132: note = IL-2 analog 94
PTSSSTKKTQLQLEHLLLDLQMILNGINNYKNPKLTRMLTFKFYMPKKATELKHLQCLEEELKPLEEVLNLAQSKNFHFEPRDVVSNINVFVFEFKGSETTFMCEYADETATIVEFLNRWITFSQSIISTLT

SEQ ID NO: 96 - protein, 132 aa, synthetic construct
  REGION 1..132: note = IL-2 analog 95
PTSSSTKKTQLQLEHLLLDLQMILNGINNYKNPKLTRMLTFKFYMPKKATELKHLQCLEEELKPLEEGLNLAQSKNFHFEPRDVVSNINVFVLELKGSETTFMCEYADETATIVEFLNRWITFSQSIISTLT

SEQ ID NO: 97 - protein, 132 aa, synthetic construct
  REGION 1..132: note = IL-2 analog 96
PTSSSTKKTQLQLEHLLLDLQMILNGINNYKNPKLTRMLTFKFYMPKKATELKHLQCLEEELKPLEEGLNLAASKNFHFEPRDVVSNINVFVLELKGSETTFMCEYADETATIVEFLNRWITFSQSIISTLT

SEQ ID NO: 98 - protein, 132 aa, synthetic construct
  REGION 1..132: note = IL-2 analog 97
PTSSSTKKTQLQLEHLLLDLQMILNGINNYKNPKLTAMLTFKFYMPKKATELKHLQCLEEELKPLEEVLNLAQSKNFHFDPRDLISNINVFVLELKGSETTFMCEYADETATIVEFLNRWITFSQSIISTLT

SEQ ID NO: 99 - protein, 132 aa, synthetic construct
  REGION 1..132: note = IL-2 analog 98
PTSSSTKKTQLQLEHLLLDLQMILNGINNYKNPKLTAMLTFKFYMPKKATELKHLQCLEEELKPLEEVLNLAQSKNFHFEPRDVISNINVFVLELKGSETTFMCEYADETATIVEFLNRWITFSQSIISTLT

SEQ ID NO: 100 - protein, 132 aa, synthetic construct
  REGION 1..132: note = IL-2 analog 99
PTSSSTKKTQLQLEHLLLDLQMILNGINNYKNPKLTAMLTFKFYMPKKATELKHLQCLEEELKPLEEVLNLAQSKNFHFEPRDLVSNINVFVLELKGSETTFMCEYADETATIVEFLNRWITFSQSIISTLT

SEQ ID NO: 101 - protein, 132 aa, synthetic construct
  REGION 1..132: note = IL-2 analog 100
PTSSSTKKTQLQLEHLLLDLQMILNGINNYKNPKLTRMLTFKFYMPKKATELKHLQCLEEELKPLEEVLNLAQSKNFHFEPRDYVSNINVFVLELKGSETTFMCEYADETATIVEFLNRWITFSQSIISTLT

SEQ ID NO: 102 - protein, 132 aa, synthetic construct
  REGION 1..132: note = IL-2 analog 101
PTSSSTKKTQLQLEHLLLDLQMILNGINNYKNPKLTRMLTFKFYMPKKATELKHLQCLEEELKPLEEVLNLAQSKNFHFEPRDLASNINVFVLELKGSETTFMCEYADETATIVEFLNRWITFSQSIISTLT

SEQ ID NO: 103 - protein, 132 aa, synthetic construct
  REGION 1..132: note = IL-2 analog 102
PTSSSTKKTQLQLEHLLLDLQMILNGINNYKNPKLTRMLTFKFYMPKKATELKHLQCLEEELKPLEEVLNLAQSKNFHFEPRDVVSNINVIVLELKGSETTFMCEYADETATIVEFLNRWITFSQSIISTLT

SEQ ID NO: 104 - protein, 132 aa, synthetic construct
  REGION 1..132: note = IL-2 analog 103
PTSSSTKKTQLQLEHLRLDLEMILNGINNYKNPKLTAMLTFKFYMPKKATELKHLQCLEEELKPLEEVLNLAQSKNFHFEPRDVVSNINVFVLELKGSETTFMCEYADETATIVEFLNRWITFSQSIISTLT

SEQ ID NO: 105 - protein, 132 aa, synthetic construct
  REGION 1..132: note = IL-2 analog 104
PTSSSTKKTQLQLEHLRLDLEMILNGINNYKNPKLTRMLTFKFYMPKKATELKHLQCLEDELKPLEEVLNLAQSKNFHFEPRDVVSNINVFVLELKGSETTFMCEYADETATIVEFLNRWITFSQSIISTLT

SEQ ID NO: 106 - protein, 132 aa, synthetic construct
  REGION 1..132: note = IL-2 analog 105
PTSSSTKKTQLQLEHLRLDLEMILNGINNYKNPKLTRMLTFKFYMPKKATELKHLQCLEEELKPLEDVLNLAQSKNFHFEPRDVVSNINVFVLELKGSETTFMCEYADETATIVEFLNRWITFSQSIISTLT

SEQ ID NO: 107 - DNA, 399 bp, synthetic construct
  misc_feature 1..399: note = IL-2 analog 1
  source 1..399: mol_type = other DNA
cctacttcaagttctacaaagaaaacacagctacaactggagcatttactgctggatttacagatgattttgaatggaattaataattacaagaatcccaaactcaccaggatgctcacatttaagttttacatgcccaagaaggccacagaactgaaacatcttcagtgtctagaagaagaactcaaacctctggaggaagtgctaaatttagctcaaagcaaaaactttcacttaagacccagggacttaatcagcaatatcaacgtaatagttctggaactaaagggatctgaaacaacattcatgtgtgaatatgctgatgagacagcaaccattgtagaatttctgaacagatggattacctttagtcaaagcatcatctcaacactgacttga

SEQ ID NO: 108 - DNA, 399 bp, synthetic construct
  misc_feature 1..399: note = IL-2 analog 2
  source 1..399: mol_type = other DNA
cctacttcaagttctacaaagaaaacacagctacaactggagcatttactgctggatttacagatgattttgaatggaattaataattacaagaatcccaaactcaccaggatgctcacatttaagttttacatgcccaagaaggccacagaactgaaacatcttcagtgtctagaagaagaactcaaacctctggaggaagtgctaaatttagctcaaagcaaaaactttcacttaagacccagggacttaatctgcaatatcaacgtaatagttctggaactaaagggatctgaaacaacattcatgtgtgaatatgctgatgagacagcaaccattgtagaatttctgaacagatggattacctttagtcaaagcatcatctcaacactgacttga

SEQ ID NO: 109 - DNA, 399 bp, synthetic construct
  misc_feature 1..399: note = IL-2 analog 3
  source 1..399: mol_type = other DNA
cctacttcaagttctacaaagaaaacacagctacaactggagcatttactgctggatttacagatgattttgaatggaattaataattactgtaatcccaaactcaccaggatgctcacatttaagttttacatgcccaagaaggccacagaactgaaacatcttcagtgtctagaagaagaactcaaacctctggaggaagtgctaaatttagctcaaagcaaaaactttcacttaagacccagggacttaatcagcaatatcaacgtaatagttctggaactaaagggatctgaaacaacattcatgtgtgaatatgctgatgagacagcaaccattgtagaatttctgaacagatggattacctttagtcaaagcatcatctcaacactgacttga

SEQ ID NO: 110 - DNA, 399 bp, synthetic construct
  misc_feature 1..399: note = IL-2 analog 4
  source 1..399: mol_type = other DNA
cctacttcaagttctacaaagaaaacacagctacaactggagcatttactgctggatttacagatgattttgaatggaattaataattacaagaatccctgtctcaccaggatgctcacatttaagttttacatgcccaagaaggccacagaactgaaacatcttcagtgtctagaagaagaactcaaacctctggaggaagtgctaaatttagctcaaagcaaaaactttcacttaagacccagggacttaatcagcaatatcaacgtaatagttctggaactaaagggatctgaaacaacattcatgtgtgaatatgctgatgagacagcaaccattgtagaatttctgaacagatggattacctttagtcaaagcatcatctcaacactgacttga

SEQ ID NO: 111 - DNA, 399 bp, synthetic construct
  misc_feature 1..399: note = IL-2 analog 5
  source 1..399: mol_type = other DNA
cctacttcaagttctacaaagaaaacacagctacaactggagcatttactgctggatttacagatgattttgaatggaattaataattacaagaatcccaaactcaccaggatgctcacattttgtttttacatgcccaagaaggccacagaactgaaacatcttcagtgtctagaagaagaactcaaacctctggaggaagtgctaaatttagctcaaagcaaaaactttcacttaagacccagggacttaatcagcaatatcaacgtaatagttctggaactaaagggatctgaaacaacattcatgtgtgaatatgctgatgagacagcaaccattgtagaatttctgaacagatggattacctttagtcaaagcatcatctcaacactgacttga

SEQ ID NO: 112 - DNA, 399 bp, synthetic construct
  misc_feature 1..399: note = IL-2 analog 6
  source 1..399: mol_type = other DNA
cctacttcaagttctacaaagaaaacacagctacaactggagcatttactgctggatttacagatgattttgaatggaattaataattacaagaatcccaaactcaccaggatgctcacatttaagttttacatgccctgtaaggccacagaactgaaacatcttcagtgtctagaagaagaactcaaacctctggaggaagtgctaaatttagctcaaagcaaaaactttcacttaagacccagggacttaatcagcaatatcaacgtaatagttctggaactaaagggatctgaaacaacattcatgtgtgaatatgctgatgagacagcaaccattgtagaatttctgaacagatggattacctttagtcaaagcatcatctcaacactgacttga

SEQ ID NO: 113 - DNA, 399 bp, synthetic construct
  misc_feature 1..399: note = IL-2 analog 7
  source 1..399: mol_type = other DNA
cctacttcaagttctacaaagaaaacacagctacaactggagcatttactgctggatttacagatgattttgaatggaattaataattacaagaatcccaaactcaccaggatgctcacatttaagttttacatgcccaagtgtgccacagaactgaaacatcttcagtgtctagaagaagaactcaaacctctggaggaagtgctaaatttagctcaaagcaaaaactttcacttaagacccagggacttaatcagcaatatcaacgtaatagttctggaactaaagggatctgaaacaacattcatgtgtgaatatgctgatgagacagcaaccattgtagaatttctgaacagatggattacctttagtcaaagcatcatctcaacactgacttga

SEQ ID NO: 114 - DNA, 399 bp, synthetic construct
  misc_feature 1..399: note = IL-2 analog 8
  source 1..399: mol_type = other DNA
cctacttcaagttctacaaagaaaacacagctacaactggagcatttactgctggatttacagatgattttgaatggaattaataattacaagaatcccaaactcaccaggatgctcacatttaagttttacatgcccaagaaggccacagaactgaaacatcttcagtgtctagaagaagaactcaaacctctggaggaagtgctaaatttagctcaaagctgtaactttcacttaagacccagggacttaatcagcaatatcaacgtaatagttctggaactaaagggatctgaaacaacattcatgtgtgaatatgctgatgagacagcaaccattgtagaatttctgaacagatggattacctttagtcaaagcatcatctcaacactgacttga

SEQ ID NO: 115 - DNA, 399 bp, synthetic construct
  misc_feature 1..399: note = IL-2 analog 9
  source 1..399: mol_type = other DNA
cctacttcaagttctacaaagaaaacacagctacaactggagcatttactgctggatttacagatgattttgaatggaattaataattacaagaatcccaaactcaccgcgatgctcacatttaagttttacatgcccaagaaggccacagaactgaaacatcttcagtgtctagaagaagaactcaaacctctggaggaagtgctaaatttagctcaaagcaaaaactttcacttaagacccagggacttaatcagcaatatcaacgtaatagttctggaactaaagggatctgaaacaacattcatgtgtgaatatgctgatgagacagcaaccattgtagaatttctgaacagatggattacctttagtcaaagcatcatctcaacactgacttga

SEQ ID NO: 116 - DNA, 399 bp, synthetic construct
  misc_feature 1..399: note = IL-2 analog 10
  source 1..399: mol_type = other DNA
cctacttcaagttctacaaagaaaacacagctacaactggagcatttactgctggatttacagatgattttgaatggaattaataattacaagaatcccaaactcaccaggatgctcacaaagaagttttacatgcccaagaaggccacagaactgaaacatcttcagtgtctagaagaagaactcaaacctctggaggaagtgctaaatttagctcaaagcaaaaactttcacttaagacccagggacttaatcagcaatatcaacgtaatagttctggaactaaagggatctgaaacaacattcatgtgtgaatatgctgatgagacagcaaccattgtagaatttctgaacagatggattacctttagtcaaagcatcatctcaacactgacttga

SEQ ID NO: 117 - DNA, 399 bp, synthetic construct
  misc_feature 1..399: note = IL-2 analog 11
  source 1..399: mol_type = other DNA
cctacttcaagttctacaaagaaaacacagctacaactggagcatttactgctggatttacagatgattttgaatggaattaataattacaagaatcccaaactcaccaggatgctcacagctaagttttacatgcccaagaaggccacagaactgaaacatcttcagtgtctagaagaagaactcaaacctctggaggaagtgctaaatttagctcaaagcaaaaactttcacttaagacccagggacttaatcagcaatatcaacgtaatagttctggaactaaagggatctgaaacaacattcatgtgtgaatatgctgatgagacagcaaccattgtagaatttctgaacagatggattacctttagtcaaagcatcatctcaacactgacttga

SEQ ID NO: 118 - DNA, 399 bp, synthetic construct
  misc_feature 1..399: note = IL-2 analog 12
  source 1..399: mol_type = other DNA
cctacttcaagttctacaaagaaaacacagctacaactggagcatttactgctggatttacagatgattttgaatggaattaataattacaagaatcccaaactcaccgcgatgctcacaaagaagttttacatgcccaagaaggccacagaactgaaacatcttcagtgtctagaagaagaactcaaacctctggaggaagtgctaaatttagctcaaagcaaaaactttcacttaagacccagggacttaatcagcaatatcaacgtaatagttctggaactaaagggatctgaaacaacattcatgtgtgaatatgctgatgagacagcaaccattgtagaatttctgaacagatggattacctttagtcaaagcatcatctcaacactgacttga

SEQ ID NO: 119 - DNA, 399 bp, synthetic construct
  misc_feature 1..399: note = IL-2 analog 13
  source 1..399: mol_type = other DNA
cctacttcaagttctacaaagaaaacacagctacaactggagcatttactgctggatttacagatgattttgaatggaattaataattacaagaatcccaaactcaccgcgatgctcacagctaagttttacatgcccaagaaggccacagaactgaaacatcttcagtgtctagaagaagaactcaaacctctggaggaagtgctaaatttagctcaaagcaaaaactttcacttaagacccagggacttaatcagcaatatcaacgtaatagttctggaactaaagggatctgaaacaacattcatgtgtgaatatgctgatgagacagcaaccattgtagaatttctgaacagatggattacctttagtcaaagcatcatctcaacactgacttga

SEQ ID NO: 120 - DNA, 399 bp, synthetic construct
  misc_feature 1..399: note = IL-2 analog 14
  source 1..399: mol_type = other DNA
cctacttcaagttctacaaagaaaacacagctacaactggagcatttactgtacgatttacagatgattttgaatggaattaataattacaagaatcccaaactcaccgcgatgctcacaaagaagttttacatgcccaagaaggccacagaactgaaacatcttcagtgtctagaagaagaactcaaacctctggaggaagtgctaaatttagctcaaagcaaaaactttcacttaagacccagggacttaatcagcaatatcaacgtaatagttctggaactaaagggatctgaaacaacattcatgtgtgaatatgctgatgagacagcaaccattgtagaatttctgaacagatggattacctttagtcaaagcatcatctcaacactgacttga

SEQ ID NO: 121 - DNA, 399 bp, synthetic construct
  misc_feature 1..399: note = IL-2 analog 15
  source 1..399: mol_type = other DNA
cctacttcaagttctacaaagaaaacacagctacaactggagcatttactgctggatttacagatgattttgaatggaattaataattacaagaatcccaaactcaccgcgatgctcacaaagaagttttacatgcccaagaaggccacagaactgaaacatcttcagtgtctagaagaagaactcaaacctctggaggaagtgctaaatttagctcaaagcaaaaactttcacttaagacccagggagttaatcagcaatatcaacgtaatagttctggaactaaagggatctgaaacaacattcatgtgtgaatatgctgatgagacagcaaccattgtagaatttctgaacagatggattacctttagtcaaagcatcatctcaacactgacttga

SEQ ID NO: 122 - DNA, 399 bp, synthetic construct
  misc_feature 1..399: note = IL-2 analog 16
  source 1..399: mol_type = other DNA
cctacttcaagttctacaaagaaaacacagctacaactggagcatttactgctggatttacagatgattttgaatggaattaataattacaagaatcccaaactcaccgcgatgctcacaaagaagttttacatgcccaagaaggccacagaactgaaacatcttcagtgtctagaagaagaactcaaacctctggaggaagtgctaaatttagctcaaagcaaaaactttcacttaagacccagggacttaatcagccaaatcaacgtaatagttctggaactaaagggatctgaaacaacattcatgtgtgaatatgctgatgagacagcaaccattgtagaatttctgaacagatggattacctttagtcaaagcatcatctcaacactgacttga

SEQ ID NO: 123 - DNA, 399 bp, synthetic construct
  misc_feature 1..399: note = IL-2 analog 17
  source 1..399: mol_type = other DNA
cctacttcaagttctacaaagaaaacacagctacaactggagcatttactgctggatttacagatgattttgaatggaattaataattacaagaatcccaaactcaccgcgatgctcacaaagaagttttacatgcccaagaaggccacagaactgaaacatcttcagtgtctagaagaagaactcaaacctctggaggaagtgctaaatttagctcaaagcaaaaactttcacttaagacccagggacttaatcagcaatatcaacacaatagttctggaactaaagggatctgaaacaacattcatgtgtgaatatgctgatgagacagcaaccattgtagaatttctgaacagatggattacctttagtcaaagcatcatctcaacactgacttga

SEQ ID NO: 124 - DNA, 399 bp, synthetic construct
  misc_feature 1..399: note = IL-2 analog 18
  source 1..399: mol_type = other DNA
cctacttcaagttctacaaagaaaacacagctacaactggagcatttactgctggatttacagatgattttgaatggaattaataattacaagaatcccaaactcaccgcgatgctcacaaagaagttttacatgcccaagaaggccacagaactgaaacatcttcagtgtctagaacaggaactcaaacctctggaggaagtgctaaatttagctcaaagcaaaaactttcacttaagacccagggacttaatcagcaatatcaacgtaatagttctggaactaaagggatctgaaacaacattcatgtgtgaatatgctgatgagacagcaaccattgtagaatttctgaacagatggattacctttagtcaaagcatcatctcaacactgacttga

SEQ ID NO: 125 - DNA, 399 bp, synthetic construct
  misc_feature 1..399: note = IL-2 analog 19
  source 1..399: mol_type = other DNA
cctacttcaagttctacaaagaaaacacagctacaactggagcatttactgctggatttacagatgattttgaatggaattaataattacaagaatcccaaactcaccgcgatgctcacaaagaagttttacatgcccaagaaggccacagaactgaaacatcttcagtgtctagaagaagaactcaaacctctggaggaagtgctaaatttagctcaaagcaaaaactttcacttagaccccagggacttaatcagcaatatcaacgtatttgttctggaactaaagggatctgaaacaacattcatgtgtgaatatgctgatgagacagcaaccattgtagaatttctgaacagatggattacctttagtcaaagcatcatctcaacactgacttga

SEQ ID NO: 126 - DNA, 399 bp, synthetic construct
  misc_feature 1..399: note = IL-2 analog 20
  source 1..399: mol_type = other DNA
cctacttcaagttctacaaagaaaacacagctacaactggagcatttactgctggatttacagatgattttgaatggaattaataattacaagaatcccaaactcaccgcgatgctcacaaagaagttttacatgcccaagaaggccacagaactgaaacatcttcagtgtctagaagaagaactcaaacctctggaggaagtgctaaatttagctcaaagcaaaaactttcacttaagacccagggacgtagtcagcaatatcaacgtatttgttctggaactaaagggatctgaaacaacattcatgtgtgaatatgctgatgagacagcaaccattgtagaatttctgaacagatggattacctttagtcaaagcatcatctcaacactgacttga

SEQ ID NO: 127 - DNA, 399 bp, synthetic construct
  misc_feature 1..399: note = IL-2 analog 21
  source 1..399: mol_type = other DNA
cctacttcaagttctacaaagaaaacacagctacaactggagcatttactgctggatttacagatgattttgaatggaattaataattacaagaatcccaaactcaccgcgatgctcacaaagaagttttacatgcccaagaaggccacagaactgaaacatcttcagtgtctagaagaagaactcaaacctctggaggaagtgctaaatttagctcaaagcaaaaactttcactttgaccccagggacgtagtcagcaatatcaacgtatttgttctggaactaaagggatctgaaacaacattcatgtgtgaatatgctgatgagacagcaaccattgtagaatttctgaacagatggattacctttagtcaaagcatcatctcaacactgacttga

SEQ ID NO: 128 - DNA, 399 bp, synthetic construct
  misc_feature 1..399: note = IL-2 analog 22
  source 1..399: mol_type = other DNA
cctacttcaagttctacaaagaaaacacaggtacaactggagcatttactgctggatttacagatgattttgaatggaattaataattacaagaatcccaaactcaccgcgatgctcacaaagaagttttacatgcccaagaaggccacagaactgaaacatcttcagtgtctagaagaagaactcaaacctctggaggaagtgctaaatttagctcaaagcaaaaactttcacttaagacccagggacttaatcagcaatatcaacgtaatagttctggaactaaagggatctgaaacaacattcatgtgtgaatatgctgatgagacagcaaccattgtagaatttctgaacagatggattacctttagtcaaagcatcatctcaacactgacttga

SEQ ID NO: 129 - DNA, 399 bp, synthetic construct
  misc_feature 1..399: note = IL-2 analog 23
  source 1..399: mol_type = other DNA
cctacttcaagttctacaaagaaaacacagtttcaactggagcatttactgctggatttacagatgattttgaatggaattaataattacaagaatcccaaactcaccgcgatgctcacaaagaagttttacatgcccaagaaggccacagaactgaaacatcttcagtgtctagaagaagaactcaaacctctggaggaagtgctaaatttagctcaaagcaaaaactttcacttaagacccagggacttaatcagcaatatcaacgtaatagttctggaactaaagggatctgaaacaacattcatgtgtgaatatgctgatgagacagcaaccattgtagaatttctgaacagatggattacctttagtcaaagcatcatctcaacactgacttga

SEQ ID NO: 130 - DNA, 399 bp, synthetic construct
  misc_feature 1..399: note = IL-2 analog 24
  source 1..399: mol_type = other DNA
cctacttcaagttctacaaagaaaacacagctacaactggagcatttactggtggatttacagatgattttgaatggaattaataattacaagaatcccaaactcaccgcgatgctcacaaagaagttttacatgcccaagaaggccacagaactgaaacatcttcagtgtctagaagaagaactcaaacctctggaggaagtgctaaatttagctcaaagcaaaaactttcacttaagacccagggacttaatcagcaatatcaacgtaatagttctggaactaaagggatctgaaacaacattcatgtgtgaatatgctgatgagacagcaaccattgtagaatttctgaacagatggattacctttagtcaaagcatcatctcaacactgacttga

SEQ ID NO: 131 - DNA, 399 bp, synthetic construct
  misc_feature 1..399: note = IL-2 analog 25
  source 1..399: mol_type = other DNA
cctacttcaagttctacaaagaaaacacagctacaactggagcatttactgttcgatttacagatgattttgaatggaattaataattacaagaatcccaaactcaccgcgatgctcacaaagaagttttacatgcccaagaaggccacagaactgaaacatcttcagtgtctagaagaagaactcaaacctctggaggaagtgctaaatttagctcaaagcaaaaactttcacttaagacccagggacttaatcagcaatatcaacgtaatagttctggaactaaagggatctgaaacaacattcatgtgtgaatatgctgatgagacagcaaccattgtagaatttctgaacagatggattacctttagtcaaagcatcatctcaacactgacttga

SEQ ID NO: 132 - DNA, 399 bp, synthetic construct
  misc_feature 1..399: note = IL-2 analog 26
  source 1..399: mol_type = other DNA
cctacttcaagttctacaaagaaaacacagctacaactggagcatttactgctggatttacagatgattttgaatggaattaataattacaagaatcccaaactcaccgcgatgctcacaaagaagttttacatgcccaagaaggccacagaactgaaacatcttcagtgtctagaagaagaactcaaacctctggaggaagtgctaaatttagctcaaagcaaaaactttcacttaagacccagggacttaatcagcaatttcaacgtaatagttctggaactaaagggatctgaaacaacattcatgtgtgaatatgctgatgagacagcaaccattgtagaatttctgaacagatggattacctttagtcaaagcatcatctcaacactgacttga

SEQ ID NO: 133 - DNA, 399 bp, synthetic construct
  misc_feature 1..399: note = IL-2 analog 27
  source 1..399: mol_type = other DNA
cctacttcaagttctacaaagaaaacacagctacaactggagcatttactgctggatttacagatgattttgaatggaattaataattacaagaatcccaaactcaccgcgatgctcacaaagaagttttacatgcccaagaaggccacagaactgaaacatcttcagtgtctagaagaagaactcaaacctctggaggaagtgctaaatttagctcaaagcaaaaactttcacttaagacccagggacttaatcagcaatatcaactttatagttctggaactaaagggatctgaaacaacattcatgtgtgaatatgctgatgagacagcaaccattgtagaatttctgaacagatggattacctttagtcaaagcatcatctcaacactgacttga

SEQ ID NO: 134 - DNA, 399 bp, synthetic construct
  misc_feature 1..399: note = IL-2 analog 28
  source 1..399: mol_type = other DNA
cctacttcaagttctacaaagaaaacacagctacaactggagcatttactgctggatttacagatgattttgaatggaattaataattacaagaatcccaaactcaccgcgatgctcacaaagaagttttacatgcccaagaaggccacagaactgaaacatcttcagtgtctagaagaagaactcaaacctctggaggaagtgctaaatttagctcaaagcaaaaactttcacttaagacccagggacttaatcagcaatatcaacgtaatagttgtggaactaaagggatctgaaacaacattcatgtgtgaatatgctgatgagacagcaaccattgtagaatttctgaacagatggattacctttagtcaaagcatcatctcaacactgacttga

SEQ ID NO: 135 - DNA, 399 bp, synthetic construct
  misc_feature 1..399: note = IL-2 analog 29
  source 1..399: mol_type = other DNA
cctacttcaagttctacaaagaaaacacagctacaactggagcatttactgctggatttacagatgattttgaatggaattaataattacaagaatcccaaactcaccgcgatgctcacaaagaagttttacatgcccaagaaggccacagaactgaaacatcttcagtgtctagaagaagaactcaaacctctggaggaagtgctaaatttagctcaaagcaaaaactttcacttaagacccagggacttaatcagcaatatcaacgtaatagttctggaactaaagggatctgaaacaacattcatgtgtgaatatgctgatgagacagcaaccattgtagaatttctgaacagatggattacctttagtacaagcatcatctcaacactgacttga

SEQ ID NO: 136 - DNA, 399 bp, synthetic construct
  misc_feature 1..399: note = IL-2 analog 30
  source 1..399: mol_type = other DNA
cctacttcaagttctacaaagaaaacacagctacaactggagcatttactgctggatttacagatgattttgaatggaattaataattacaagaatcccaaactcaccgcgatgctcacatttaagttttacatgcccaagaaggccacagaactgaaacatcttcagtgtctagaagaagaactcaaacctctggaggaagtgctaaatttagctcaaagcaaaaactttcacttagaccccagggacttaatcagcaatatcaacgtatttgttctggaactaaagggatctgaaacaacattcatgtgtgaatatgctgatgagacagcaaccattgtagaatttctgaacagatggattacctttagtcaaagcatcatctcaacactgacttga

SEQ ID NO: 137 - DNA, 399 bp, synthetic construct
  misc_feature 1..399: note = IL-2 analog 31
  source 1..399: mol_type = other DNA
cctacttcaagttctacaaagaaaacacagctacaactggagcatttactgctggatttacagatgattttgaatggaattaataattacaagaatcccaaactcaccgcgatgctcacatttaagttttacatgcccaagaaggccacagaactgaaacatcttcagtgtctagaagaagaactcaaacctctggaggaagtgctaaatttagctcaaagcaaaaactttcacttaagacccagggagttaatcagcaatatcaacgtaatagttctggaactaaagggatctgaaacaacattcatgtgtgaatatgctgatgagacagcaaccattgtagaatttctgaacagatggattacctttagtcaaagcatcatctcaacactgacttga

SEQ ID NO: 138 - DNA, 399 bp, synthetic construct
  misc_feature 1..399: note = IL-2 analog 32
  source 1..399: mol_type = other DNA
cctacttcaagttctacaaagaaaacacagctacaactggagcatttactgctggatttacagatgattttgaatggaattaataattacaagaatcccaaactcaccgcgatgctcacatttaagttttacatgcccaagaaggccacagaactgaaacatcttcagtgtctagaagaagaactcaaacctctggaggaagtgctaaatttagctcaaagcaaaaactttcacttagaccccagggagttaatcagcaatatcaacgtatttgttctggaactaaagggatctgaaacaacattcatgtgtgaatatgctgatgagacagcaaccattgtagaatttctgaacagatggattacctttagtcaaagcatcatctcaacactgacttga

SEQ ID NO: 139 - DNA, 399 bp, synthetic construct
  misc_feature 1..399: note = IL-2 analog 33
  source 1..399: mol_type = other DNA
cctacttcaagttctacaaagaaaacacagctacaactggagcatttactgctggatttacagatgattttgaatggaattaataattacaagaatcccaaactcaccgcgatgctcacatttaagttttacatgcccaagaaggccacagaactgaaacatcttcagtgtctagaagaagaactcaaacctctggaggaagtgctaaatttagctcaaagcaaaaactttcactttagacccagggacttaatcagcaatatcaacgtaatagttctggaactaaagggatctgaaacaacattcatgtgtgaatatgctgatgagacagcaaccattgtagaatttctgaacagatggattacctttagtcaaagcatcatctcaacactgacttga

SEQ ID NO: 140 - DNA, 399 bp, synthetic construct
  misc_feature 1..399: note = IL-2 analog 34
  source 1..399: mol_type = other DNA
cctacttcaagttctacaaagaaaacacagctacaactggagcatttactgctggatttacagatgattttgaatggaattaataattacaagaatcccaaactcaccgcgatgctcacatttaagttttacatgcccaagaaggccacagaactgaaacatcttcagtgtctagaagaagaactcaaacctctggaggaagtgctaaatttagctcaaagcaaaaactttcactttagacccagggagttaatcagcaatatcaacgtaatagttctggaactaaagggatctgaaacaacattcatgtgtgaatatgctgatgagacagcaaccattgtagaatttctgaacagatggattacctttagtcaaagcatcatctcaacactgacttga

SEQ ID NO: 141 - DNA, 399 bp, synthetic construct
  misc_feature 1..399: note = IL-2 analog 35
  source 1..399: mol_type = other DNA
cctacttcaagttctacaaagaaaacacagctacaactggagcatttactgctggatttacagatgattttgaatggaattaataattacaagaatcccaaactcaccgcgatgctcacatttaagttttacatgcccaagaaggccacagaactgaaacatcttcagtgtctagaagaagaactcaaacctctggaggaagtgctaaatttagctcaaagcaaaaactttcacttaagacccagggacttaatcagcaatatcaacgtaatagttttcgaatttaagggatctgaaacaacattcatgtgtgaatatgctgatgagacagcaaccattgtagaatttctgaacagatggattacctttagtcaaagcatcatctcaacactgacttga

SEQ ID NO: 142 - DNA, 399 bp, synthetic construct
  misc_feature 1..399: note = IL-2 analog 36
  source 1..399: mol_type = other DNA
cctacttcaagttctacaaagaaaacacagctacaactggagcatttactgctggatttacagatgattttgaatggaattaataattacaagaatcccaaactcaccgcgatgctcacatttaagttttacatgcccaagaaggccacagaactgaaacatcttcagtgtctagaagaagaactcaaacctctggaggaagtgctaaatttagctcaaagcaaaaactttcacttaagacccagggacttaatcagcaatatcaacgtaatagttttcgaagtaaagggatctgaaacaacattcatgtgtgaatatgctgatgagacagcaaccattgtagaatttctgaacagatggattacctttagtcaaagcatcatctcaacactgacttga

SEQ ID NO: 143 - DNA, 399 bp, synthetic construct
  misc_feature 1..399: note = IL-2 analog 37
  source 1..399: mol_type = other DNA
cctacttcaagttctacaaagaaaacacagctacaactggagcatttactgctggatttacagatgattttgaatggaattaataattacaagaatcccaaactcaccgcgatgctcacaaagaagttttacatgcccaagaaggccacagaactgaaacatcttcagtgtctagaagaagaactcaaacctctggaggaagtgctaaatttagctcaaagcaaaaactttcacttagaccccagggacttaatcagcaatatcaacgtattagttctggaactaaagggatctgaaacaacattcatgtgtgaatatgctgatgagacagcaaccattgtagaatttctgaacagatggattacctttagtcaaagcatcatctcaacactgacttga

SEQ ID NO: 144 - DNA, 399 bp, synthetic construct
  misc_feature 1..399: note = IL-2 analog 38
  source 1..399: mol_type = other DNA
cctacttcaagttctacaaagaaaacacagctacaactggagcatttactgctggatttacagatgattttgaatggaattaataattacaagaatcccaaactcaccgcgatgctcacaaagaagttttacatgcccaagaaggccacagaactgaaacatcttcagtgtctagaagaagaactcaaacctctggaggaagtgctaaatttagctcaaagcaaaaactttcacttagaccccagggacttaatcagcaatatcaacgtatttgttttcgaatttaagggatctgaaacaacattcatgtgtgaatatgctgatgagacagcaaccattgtagaatttctgaacagatggattacctttagtcaaagcatcatctcaacactgacttga

SEQ ID NO: 145 - DNA, 399 bp, synthetic construct
  misc_feature 1..399: note = IL-2 analog 39
  source 1..399: mol_type = other DNA
cctacttcaagttctacaaagaaaacacagctacaactggagcatttactgctggatttacagatgattttgaatggaattaataattacaagaatcccaaactcaccgcgatgctcacaaagaagttttacatgcccaagaaggccacagaactgaaacatcttcagtgtctagaagaagaactcaaacctctggaggaagtgctaaatttagctcaaagcaaaaactttcacttagaccccagggacttaatcagcaatatcaacgtatttgttttcgaagtaaagggatctgaaacaacattcatgtgtgaatatgctgatgagacagcaaccattgtagaatttctgaacagatggattacctttagtcaaagcatcatctcaacactgacttga

SEQ ID NO: 146 - DNA, 399 bp, synthetic construct
  misc_feature 1..399: note = IL-2 analog 40
  source 1..399: mol_type = other DNA
cctacttcaagttctacaaagaaaacacagctacaactggagcatttactgctggatttacagatgattttgaatggaattaataattacaagaatcccaaactcaccgcgatgctcacaaagaagttttacatgcccaagaaggccacagaactgaaacatcttcagtgtctagaagaagaactcaaacctctggaggaagtgctaaatttagctcaaagcaaaaactttcacttagaccccagggacttaatcagcaatatcaacgtatttgttttcgaaattaagggatctgaaacaacattcatgtgtgaatatgctgatgagacagcaaccattgtagaatttctgaacagatggattacctttagtcaaagcatcatctcaacactgacttga

SEQ ID NO: 147 - DNA, 399 bp, synthetic construct
  misc_feature 1..399: note = IL-2 analog 41
  source 1..399: mol_type = other DNA
cctacttcaagttctacaaagaaaacacagctacaactggagcatttactgctggatttacagatgattttgaatggaattaataattacaagaatcccaaactcaccaggatgctcacatttaagttttacatgcccaagaaggccacagaactgaaacatcttcagtgtctagaagaagaactcaaacctctggaggaagtgctaaatttagctcaaagcaaaaactttcactttgaccccagggacgtagtcagcaatatcaacgtatttgttctggaactaaagggatctgaaacaacattcatgtgtgaatatgctgatgagacagcaaccattgtagaatttctgaacagatggattacctttagtcaaagcatcatctcaacactgacttga

SEQ ID NO: 148 - DNA, 399 bp, synthetic construct
  misc_feature 1..399: note = IL-2 analog 42
  source 1..399: mol_type = other DNA
cctacttcaagttctacaaagaaaacacagctacaactggagcatttactgctggatttacagatgattttgaatggaattaataattacaagaatcccaaactcaccgcgatgctcacaaagaagttttacatgcccaagaaggccacagaactgaaacatcttcagtgtctagaagaagaactcaaacctctggaggaagtgctaaatttagctcaaagcaaaaactttcacttagaacccagggacttaatcagcaatatcaacgtatttgttctggaactaaagggatctgaaacaacattcatgtgtgaatatgctgatgagacagcaaccattgtagaatttctgaacagatggattacctttagtcaaagcatcatctcaacactgacttga

SEQ ID NO: 149 - DNA, 399 bp, synthetic construct; identical to SEQ ID NO: 143
  misc_feature 1..399: note = IL-2 analog 43
  source 1..399: mol_type = other DNA

SEQ ID NO: 150 - DNA, 399 bp, synthetic construct
  misc_feature 1..399: note = IL-2 analog 44
  source 1..399: mol_type = other DNA
cctacttcaagttctacaaagaaaacacagctacaactggagcatttactgctggatttacagatgattttgaatggaattaataattacaagaatcccaaactcaccgcgatgctcacaaagaagttttacatgcccaagaaggccacagaactgaaacatcttcagtgtctagaagaagaactcaaacctctggaggaagtgctaaatttagctcaaagcaaaaactttcacttagaccccagggtcttaatcagcaatatcaacgtatttgttctggaactaaagggatctgaaacaacattcatgtgtgaatatgctgatgagacagcaaccattgtagaatttctgaacagatggattacctttagtcaaagcatcatctcaacactgacttga

SEQ ID NO: 151 - DNA, 399 bp, synthetic construct
  misc_feature 1..399: note = IL-2 analog 45
  source 1..399: mol_type = other DNA
cctacttcaagttctacaaagaaaacacagctacaactggagcatttactgctggatttacagatgattttgaatggaattaataattacaagaatcccaaactcaccgcgatgctcacaaagaagttttacatgcccaagaaggccacagaactgaaacatcttcagtgtctagaagaagaactcaaacctctggaggaagtgctaaatttagctcaaagcaaaaactttcacttagaccccaggttcttaatcagcaatatcaacgtatttgttctggaactaaagggatctgaaacaacattcatgtgtgaatatgctgatgagacagcaaccattgtagaatttctgaacagatggattacctttagtcaaagcatcatctcaacactgacttga

SEQ ID NO: 152 - DNA, 399 bp, synthetic construct
  misc_feature 1..399: note = IL-2 analog 46
  source 1..399: mol_type = other DNA
cctacttcaagttctacaaagaaaacacagctacaactggagcatttactgctggttttacagatgattttgaatggaattaataattacaagaatcccaaactcaccgcgatgctcacaaagaagttttacatgcccaagaaggccacagaactgaaacatcttcagtgtctagaagaagaactcaaacctctggaggaagtgctaaatttagctcaaagcaaaaactttcacttagaccccagggacttaatcagcaatatcaacgtatttgttctggaactaaagggatctgaaacaacattcatgtgtgaatatgctgatgagacagcaaccattgtagaatttctgaacagatggattacctttagtcaaagcatcatctcaacactgacttga

SEQ ID NO: 153 - DNA, 399 bp, synthetic construct
  misc_feature 1..399: note = IL-2 analog 47
  source 1..399: mol_type = other DNA
cctacttcaagttctacaaagaaaacacagctacaactggagcatttactgctgtttttacagatgattttgaatggaattaataattacaagaatcccaaactcaccgcgatgctcacaaagaagttttacatgcccaagaaggccacagaactgaaacatcttcagtgtctagaagaagaactcaaacctctggaggaagtgctaaatttagctcaaagcaaaaactttcacttagaccccagggacttaatcagcaatatcaacgtatttgttctggaactaaagggatctgaaacaacattcatgtgtgaatatgctgatgagacagcaaccattgtagaatttctgaacagatggattacctttagtcaaagcatcatctcaacactgacttga

SEQ ID NO: 154 - DNA, 399 bp, synthetic construct
  misc_feature 1..399: note = IL-2 analog 48
  source 1..399: mol_type = other DNA
cctacttcaagttctacaaagaaaacacagctacaactggagcatttactgctggatttacagatgattttgaatggaattaataattacaagaatcccaaactcaccgcgatgctcacaaagaagttttacatgcccaagaaggccacagaactgaaacatcttcagtgtctagaagaagaactcaaacctctggaggaagtgctaaatttagctcaaagcaaaaactttcacttagaccccagggacttaatcagcgttatcaacgtatttgttctggaactaaagggatctgaaacaacattcatgtgtgaatatgctgatgagacagcaaccattgtagaatttctgaacagatggattacctttagtcaaagcatcatctcaacactgacttga

SEQ ID NO: 155 - DNA, 399 bp, synthetic construct
  misc_feature 1..399: note = IL-2 analog 49
  source 1..399: mol_type = other DNA
cctacttcaagttctacaaagaaaacacagctacaactggagcatttactgctggatttacagatgattttgaatggaattaataattacaagaatcccaaactcaccgcgatgctcacaaagaagttttacatgcccaagaaggccacagaactgaaacatcttcagtgtctagaagaagaactcaaacctctggaggaagtgctaaatttagctcaaagcaaaaactttcacttagaccccagggacttaatcagctttatcaacgtatttgttctggaactaaagggatctgaaacaacattcatgtgtgaatatgctgatgagacagcaaccattgtagaatttctgaacagatggattacctttagtcaaagcatcatctcaacactgacttga

SEQ ID NO: 156 - DNA, 399 bp, synthetic construct
  misc_feature 1..399: note = IL-2 analog 50
  source 1..399: mol_type = other DNA
cctacttcaagttctacaaagaaaacacagctacaactggagcatttactgctggatttacagatgattttgaatggaattaataattacaagaatcccaaactcaccaggatgctcacaaagaagttttacatgcccaagaaggccacagaactgaaacatcttcagtgtctagaagaagaactcaaacctctggaggaagtgctaaatttagctcaaagcaaaaactttcactttgaccccagggacgtagtcagcaatatcaacgtatttgttctggaactaaagggatctgaaacaacattcatgtgtgaatatgctgatgagacagcaaccattgtagaatttctgaacagatggattacctttagtcaaagcatcatctcaacactgacttga

SEQ ID NO: 157 - DNA, 399 bp, synthetic construct
  misc_feature 1..399: note = IL-2 analog 51
  source 1..399: mol_type = other DNA
cctacttcaagttctacaaagaaaacacagctacaactggagcatttactgctggatttacagatgattttgaatggaattaataattacaagaatcccaaactcaccaggatgctcacatttaagttttacatgcccaagaaggccacagaactgaaacatcttcagtgtctagaacaggaactcaaacctctggaggaagtgctaaatttagctcaaagcaaaaactttcacttagaccccagggacttaatcagcaatatcaacgtatttgttctggaactaaagggatctgaaacaacattcatgtgtgaatatgctgatgagacagcaaccattgtagaatttctgaacagatggattacctttagtcaaagcatcatctcaacactgacttga

SEQ ID NO: 158 - DNA, 399 bp, synthetic construct
  misc_feature 1..399: note = IL-2 analog 52
  source 1..399: mol_type = other DNA
cctacttcaagttctacaaagaaaacacagctacaactggagcatttactgctggatttacagatgattttgaatggaattaataattacaagaatcccaaactcaccgcgatgctcacaaagaagttttacatgcccaagaaggccacagaactgaaacatcttcagtgtctagaagaagaactcaaacctctggaggaagtgctaaatttagctcaaagcaaaaactttcactttgaccccagggacttaatcagcaatatcaacgtatttgttctggaactaaagggatctgaaacaacattcatgtgtgaatatgctgatgagacagcaaccattgtagaatttctgaacagatggattacctttagtcaaagcatcatctcaacactgacttga

SEQ ID NO: 159 - DNA, 399 bp, synthetic construct
  misc_feature 1..399: note = IL-2 analog 53
  source 1..399: mol_type = other DNA
cctacttcaagttctacaaagaaaacacagctacaactggagcatttactgctggatttacagatgattttgaatggaattaataattacaagaatcccaaactcaccgcgatgctcacaaagaagttttacatgcccaagaaggccacagaactgaaacatcttcagtgtctagaagaagaactcaaacctctggaggaagtgctaaatttagctcaaagcaaaaactttcactttgaccccagggagttaatcagcaatatcaacgtatttgttctggaactaaagggatctgaaacaacattcatgtgtgaatatgctgatgagacagcaaccattgtagaatttctgaacagatggattacctttagtcaaagcatcatctcaacactgacttga

SEQ ID NO: 160 - DNA, 399 bp, synthetic construct
  misc_feature 1..399: note = IL-2 analog 54
  source 1..399: mol_type = other DNA
cctacttcaagttctacaaagaaaacacagctacaactggagcatttactgctggatttacagatgattttgaatggaattaataattacaagaatcccaaactcaccgcgatgctcacaaagaagttttacatgcccaagaaggccacagaactgaaacatcttcagtgtctagaagaagaactcaaacctctggaggaagtgctaaatttagctcacagcaaaaactttcacttagaccccagggacttaatcagcaatatcaacgtatttgttctggaactaaagggatctgaaacaacattcatgtgtgaatatgctgatgagacagcaaccattgtagaatttctgaacagatggattacctttagtcaaagcatcatctcaacactgacttga

SEQ ID NO: 161 - DNA, 399 bp, synthetic construct
  misc_feature 1..399: note = IL-2 analog 55
  source 1..399: mol_type = other DNA
cctacttcaagttctacaaagaaaacacagctacaactggagcatttactgctggatttacagatgattttgaatggaattaataattacaagaatcccaaactcaccgcgatgctcacaaagaagttttacatgcccaagaaggccacagaactgaaacatcttcagtgtctagaagaagaactcaaacctctggaggaagtgctaaatttagctcacagcaaaaactttcactttgaccccagggacttaatcagcaatatcaacgtatttgttctggaactaaagggatctgaaacaacattcatgtgtgaatatgctgatgagacagcaaccattgtagaatttctgaacagatggattacctttagtcaaagcatcatctcaacactgacttga

SEQ ID NO: 162 - DNA, 399 bp, synthetic construct
  misc_feature 1..399: note = IL-2 analog 56
  source 1..399: mol_type = other DNA
cctacttcaagttctacaaagaaaacacagctacaactggagcatttactgctggatttacagatgattttgaatggaattaataattacaagaatcccaaactcaccgcgatgctcacaaagaagtttgccatgcccaagaaggccacagaactgaaacatcttcagtgtctagaagaagaactcaaacctctggaggaagtgctaaatttagctcacagcaaaaactttcacttagaccccagggacttaatcagcaatatcaacgtatttgttctggaactaaagggatctgaaacaacattcatgtgtgaatatgctgatgagacagcaaccattgtagaatttctgaacagatggattacctttagtcaaagcatcatctcaacactgacttga

SEQ ID NO: 163 - DNA, 399 bp, synthetic construct
  misc_feature 1..399: note = IL-2 analog 57
  source 1..399: mol_type = other DNA
cctacttcaagttctacaaagaaaacacagctacaactggagcatttactgctggatttacagatgattttgaatggaattaataattacaagaatcccaaactcaccgcgatgctcacaaagaagtttgccatgcccaagaaggccacagaactgaaacatcttcagtgtctagaagaagaactcaaacctctggaggaagtgctaaatttagctcacagcaaaaactttcactttgaccccagggacttaatcagcaatatcaacgtatttgttctggaactaaagggatctgaaacaacattcatgtgtgaatatgctgatgagacagcaaccattgtagaatttctgaacagatggattacctttagtcaaagcatcatctcaacactgacttga

SEQ ID NO: 164 - DNA, 399 bp, synthetic construct
  misc_feature 1..399: note = IL-2 analog 58
  source 1..399: mol_type = other DNA
cctacttcaagttctacaaagaaaacacagctacaactggagcatttactgctggatttacagatgattttgaatggaattaataattacaagaatcccaaactcaccgcgatgctcacaaagaagttttacatgcccaagaaggccacagaactgaaacatcttcagtgtctagaagaagaactcaaacctctggaggaagtgctaaatttagctcaaagcaaaaactttcactttgaccccagggacgctgccagcaatatcaacgtatttgttctggaactaaagggatctgaaacaacattcatgtgtgaatatgctgatgagacagcaaccattgtagaatttctgaacagatggattacctttagtcaaagcatcatctcaacactgacttga

SEQ ID NO: 165 - DNA, 399 bp, synthetic construct
  misc_feature 1..399: note = IL-2 analog 59
  source 1..399: mol_type = other DNA
cctacttcaagttctacaaagaaaacacagctacaactggagcatttactgctggatttacagatgattttgaatggaattaataattacaagaatcccaaactcaccgcgatgctcacaaagaagttttacatgcccaagaaggccacagaactgaaacatcttcagtgtctagaagaagaactcaaacctctggaggaagtgctaaatttagctcaaagcaaaaactttcactttgaccccagggacgctgccagcaatatcaacgtatatgttctggaactaaagggatctgaaacaacattcatgtgtgaatatgctgatgagacagcaaccattgtagaatttctgaacagatggattacctttagtcaaagcatcatctcaacactgacttga

SEQ ID NO: 166 - DNA, 399 bp, synthetic construct
  misc_feature 1..399: note = IL-2 analog 60
  source 1..399: mol_type = other DNA
cctacttcaagttctacaaagaaaacacagctacaactggagcatttactgctggatttacagatgattttgaatggaattaataattacaagaatcccaaactcaccgcgatgctcacaaagaagtttgccatgcccaagaaggccacagaactgaaacatcttcagtgtctagaagaagaactcaaacctctggaggaagtgctaaatttagctcaaagcaaaaactttcactatagacccagggacgctgccagcaatatcaacgtatatgttctggaactaaagggatctgaaacaacattcatgtgtgaatatgctgatgagacagcaaccattgtagaatttctgaacagatggattacctttagtcaaagcatcatctcaacactgacttga

SEQ ID NO: 167 - DNA, 399 bp, synthetic construct
  misc_feature 1..399: note = IL-2 analog 61
  source 1..399: mol_type = other DNA
cctacttcaagttctacaaagaaaacacagctacaactggagcatttactgctggatttacagatgattttgaatggaattaataattacaagaatcccaaactcaccgcgatgctcacaaagaagttttacatgcccaagaaggccacagaactgaaacatcttcagtgtctagaagaagaactcaaacctctggaggaagtgctaaatttagctcaaagcaaaaactttcactatgaccccagggacggtgttagcaatatcaacgtatatgttctggaactaaagggatctgaaacaacattcatgtgtgaatatgctgatgagacagcaaccattgtagaatttctgaacagatggattacctttagtcaaagcatcatctcaacactgacttga

SEQ ID NO: 168 - DNA, 399 bp, synthetic construct
  misc_feature 1..399: note = IL-2 analog 62
  source 1..399: mol_type = other DNA
cctacttcaagttctacaaagaaaacacagctacaactggagcatttactgctggatttacagatgattttgaatggaattaataattacaagaatcccaaactcaccgcgatgctcacaaagaagttttacatgcccaagaaggccacagaactgaaacatcttcagtgtctagaagaagaactcaaacctctggaggaagtgctaaatttagctcaaagcaaaaactttcactgggaacccagggacggagccagcaatatcaacgtatttgttctggaactaaagggatctgaaacaacattcatgtgtgaatatgctgatgagacagcaaccattgtagaatttctgaacagatggattacctttagtcaaagcatcatctcaacactgacttga

SEQ ID NO: 169 - DNA, 399 bp, synthetic construct
  misc_feature 1..399: note = IL-2 analog 63
  source 1..399: mol_type = other DNA
cctacttcaagttctacaaagaaaacacagctacaactggagcatttactgctggatttacagatgattttgaatggaattaataattacaagaatcccaaactcaccgcgatgctcacaaagaagttttacatgcccaagaaggccacagaactgaaacatcttcagtgtctagaagaagaactcaaacctctggaggaagtgctaaatttagctcaaagcaaaaactttcacgacgaacccagggacacaggcagcaatatcaacgtatttgttctggaactaaagggatctgaaacaacattcatgtgtgaatatgctgatgagacagcaaccattgtagaatttctgaacagatggattacctttagtcaaagcatcatctcaacactgacttga

SEQ ID NO: 170 - DNA, 399 bp, synthetic construct
  misc_feature 1..399: note = IL-2 analog 64
  source 1..399: mol_type = other DNA
cctacttcaagttctacaaagaaaacacagctacaactggagcatttactgctggatttacagatgattttgaatggaattaataattacaagaatcccaaactcaccgcgatgctcacaaagaagttttacatgcccaagaaggccacagaactgaaacatcttcagtgtctagaagaagaactcaaacctctggaggaagtgctaaatttagctcaaagcaaaaactttcactacaaccccagggacgtagtcagcaatatcaacgtatttgttctggaactaaagggatctgaaacaacattcatgtgtgaatatgctgatgagacagcaaccattgtagaatttctgaacagatggattacctttagtcaaagcatcatctcaacactgacttga

SEQ ID NO: 171 - DNA, 399 bp, synthetic construct
  misc_feature 1..399: note = IL-2 analog 65
  source 1..399: mol_type = other DNA
cctacttcaagttctacaaagaaaacacagctacaactggagcatttactgctggatttacagatgattttgaatggaattaataattacaagaatcccaaactcaccgcgatgctcacaaagaagttttacatgcccaagaaggccacagaactgaaacatcttcagtgtctagaagaagaactcaaacctctggaggaagtgctaaatttagctcaaagcaaaaactttcactacgaacccagggacgtagtcagcaatatcaacgtatttgttctggaactaaagggatctgaaacaacattcatgtgtgaatatgctgatgagacagcaaccattgtagaatttctgaacagatggattacctttagtcaaagcatcatctcaacactgacttga

SEQ ID NO: 172 - DNA, 399 bp, synthetic construct
  misc_feature 1..399: note = IL-2 analog 66
  source 1..399: mol_type = other DNA
cctacttcaagttctacaaagaaaacacagctacaactggagcatttactgctggatttacagatgattttgaatggaattaataattacaagaatcccaaactcaccgcgatgctcacaaagaagttttacatgcccaagaaggccacagaactgaaacatcttcagtgtctagaagaagaactcaaacctctggaggaagtgctaaatttagctcaaagcaaaaactttcacttcgaacccagggacttcgtcagcaatatcaacgtatttgttctggaactaaagggatctgaaacaacattcatgtgtgaatatgctgatgagacagcaaccattgtagaatttctgaacagatggattacctttagtcaaagcatcatctcaacactgacttga

SEQ ID NO: 173 - DNA, 399 bp, synthetic construct
  misc_feature 1..399: note = IL-2 analog 67
  source 1..399: mol_type = other DNA
cctacttcaagttctacaaagaaaacacagctacaactggagcatttactgctggatttacagatgattttgaatggaattaataattacaagaatcccaaactcaccgcgatgctcacaaagaagttttacatgcccaagaaggccacagaactgaaacatcttcagtgtctagaagaagaactcaaacctctggaggaagtgctaaatttagctcaaagcaaaaactttcactatgaccccagggacttcgtcagcaatatcaacgtatgggttctggacctaaagggatctgaaacaacattcatgtgtgaatatgctgatgagacagcaaccattgtagaatttctgaacagatggattacctttagtcaaagcatcatctcaacactgacttga

SEQ ID NO: 174 - DNA, 399 bp, synthetic construct
  misc_feature 1..399: note = IL-2 analog 68
  source 1..399: mol_type = other DNA
cctacttcaagttctacaaagaaaacacagctacaactggagcatttactgctggatttacagatgattttgaatggaattaataattacaagaatcccaaactcaccgcgatgctcacaaagaagttttacatgcccaagaaggccacagaactgaaacatcttcagtgtctagaagaagaactcaaacctctggaggaagtgctaaatttagctcaaagcaaaaactttcacttcgaacccagggacatagtcagcaatatcaacgaattcgttctggaactaaagggatctgaaacaacattcatgtgtgaatatgctgatgagacagcaaccattgtagaatttctgaacagatggattacctttagtcaaagcatcatctcaacactgacttga

SEQ ID NO: 175 - DNA, 399 bp, synthetic construct
  misc_feature 1..399: note = IL-2 analog 69
  source 1..399: mol_type = other DNA
cctacttcaagttctacaaagaaaacacagctacaactggagcatttactgctggatttacagatgattttgaatggaattaataattacaagaatcccaaactcaccgcgatgctcacaaagaagttttacatgcccaagaaggccacagaactgaaacatcttcagtgtctagaagaagaactcaaacctctggaggaagtgctaaatttagctcaaagcaaaaactttcactacgaacccagggacttcctcagcaatatcaacgaatgggttctggacctaaagggatctgaaacaacattcatgtgtgaatatgctgatgagacagcaaccattgtagaatttctgaacagatggattacctttagtcaaagcatcatctcaacactgacttga

SEQ ID NO: 176 - DNA, 399 bp, synthetic construct
  misc_feature 1..399: note = IL-2 analog 70
  source 1..399: mol_type = other DNA
cctacttcaagttctacaaagaaaacacagctacaactggagcatttactgctggatttacagatgattttgaatggaattaataattacaagaatcccaaactcaccgcgatgctcacaaagaagttttacatgcccaagaaggccacagaactgaaacatcttcagtgtctagaagaagaactcaaacctctggaggaagtgctaaatttagctcaaagcaaaaactttcactatgaccccagggacgtagtcagcaatatcaacgtatttgttctggaactaaagggatctgaaacaacattcatgtgtgaatatgctgatgagacagcaaccattgtagaatttctgaacagatggattacctttagtcaaagcatcatctcaacactgacttga

SEQ ID NO: 177 - DNA, 399 bp, synthetic construct
  misc_feature 1..399: note = IL-2 analog 71
  source 1..399: mol_type = other DNA
cctacttcaagttctacaaagaaaacacagctacaactggagcatttactgctggatttacagatgattttgaatggaattaataattacaagaatcccaaactcaccgcgatgctcacaaagaagttttacatgcccaagaaggccacagaactgaaacatcttcagtgtctagaagaagaactcaaacctctggaggaagtgctaaatttagctcaaagcaaaaactttcacttcgaacccagggacgtagtcagcaatatcaacgtatttgttctggaactaaagggatctgaaacaacattcatgtgtgaatatgctgatgagacagcaaccattgtagaatttctgaacagatggattacctttagtcaaagcatcatctcaacactgacttga

SEQ ID NO: 178 - DNA, 399 bp, synthetic construct
  misc_feature 1..399: note = IL-2 analog 72
  source 1..399: mol_type = other DNA
cctacttcaagttctacaaagaaaacacagctacaactggagcatttactgctggatttacagatgattttgaatggaattaataattacaagaatcccaaactcaccgcgatgctcacaaagaagttttacatgcccaagaaggccacagaactgaaacatcttcagtgtctagaagaagaactcaaacctctggaggaagtgctaaatttagctcaaagcaaaaactttcactttgaccccagggacgtaggcagcaatatcaacgtatttgttctggaactaaagggatctgaaacaacattcatgtgtgaatatgctgatgagacagcaaccattgtagaatttctgaacagatggattacctttagtcaaagcatcatctcaacactgacttga

SEQ ID NO: 179 - DNA, 399 bp, synthetic construct
  misc_feature 1..399: note = IL-2 analog 73
  source 1..399: mol_type = other DNA
cctacttcaagttctacaaagaaaacacagctacaactggagcatttactgctggatttacagatgattttgaatggaattaataattacaagaatcccaaactcaccgcgatgctcacaaagaagttttacatgcccaagaaggccacagaactgaaacatcttcagtgtctagaagaagaactcaaacctctggaggaagtgctaaatttagctcaaagcaaaaactttcactttgaccccagggactgggtcagcaatatcaacgtatttgttctggaactaaagggatctgaaacaacattcatgtgtgaatatgctgatgagacagcaaccattgtagaatttctgaacagatggattacctttagtcaaagcatcatctcaacactgacttga

SEQ ID NO: 180 - DNA, 399 bp, synthetic construct
  misc_feature 1..399: note = IL-2 analog 74
  source 1..399: mol_type = other DNA
cctacttcaagttctacaaagaaaacacagctacaactggagcatttactgctggatttacagatgattttgaatggaattaataattacaagaatcccaaactcaccgatatgctcacaaagaagttttacatgcccaagaaggccacagaactgaaacatcttcagtgtctagaagaagaactcaaacctctggaggaagtgctaaatttagctcaaagcaaaaactttcactatgaccccagggacgtagtcagcaatatcaacgtatttgttctggaactaaagggatctgaaacaacattcatgtgtgaatatgctgatgagacagcaaccattgtagaatttctgaacagatggattacctttagtcaaagcatcatctcaacactgacttga

SEQ ID NO: 181 - DNA, 399 bp, synthetic construct
  misc_feature 1..399: note = IL-2 analog 75
  source 1..399: mol_type = other DNA
cctacttcaagttctacaaagaaaacacagctacaactggagcatttactgctggatttacagatgattttgaatggaattaataattacaagaatcccaaactcaccgcgatgctcacaaagaagtttgccatgcccaagaaggccacagaactgaaacatcttcagtgtctagaagaagaactcaaacctctggaggaagtgctaaatttagctcaaagcaaaaactttcacttcgaacccagggacgtagtcagcaatatcaacgtatttgttctggaactaaagggatctgaaacaacattcatgtgtgaatatgctgatgagacagcaaccattgtagaatttctgaacagatggattacctttagtcaaagcatcatctcaacactgacttga

SEQ ID NO: 182 - DNA, 399 bp, synthetic construct
  misc_feature 1..399: note = IL-2 analog 76
  source 1..399: mol_type = other DNA
cctacttcaagttctacaaagaaaacacagctacaactggagcatttactgctggatttacagatgattttgaatggaattaataattacaagaatcccaaactcaccgcgatgctcacaaagcagttttacatgcccaagaaggccacagaactgaaacatcttcagtgtctagaacgggaactcaaacctctggaggaagtgctaaatttagctcaaagcaaaaactttcactttgaccccagggacgtaggcagcaatatcaacgtatttgttctggaactaaagggatctgaaacaacattcatgtgtgaatatgctgatgagacagcaaccattgtagaatttctgaacagatggattacctttagtcaaagcatcatctcaacactgacttga

SEQ ID NO: 183 - DNA, 399 bp, synthetic construct
  misc_feature 1..399: note = IL-2 analog 77
  source 1..399: mol_type = other DNA
cctacttcaagttctacaaagaaaacacagctacaactggagcatttactgctggatttacagatgattttgaatggaattaataattacaagaatcccaaactcaccgcgatgctcacaaaggagttttacatgcccaagaaggccacagaactgaaacatcttcagtgtctagaacgggaactcaaacctctggaggaagtgctaaatttagctcaaagcaaaaactttcactttgaccccagggactgggtcagcaatatcaacgtatttgttctggaactaaagggatctgaaacaacattcatgtgtgaatatgctgatgagacagcaaccattgtagaatttctgaacagatggattacctttagtcaaagcatcatctcaacactgacttga

SEQ ID NO: 184 - DNA, 399 bp, synthetic construct
  misc_feature 1..399: note = IL-2 analog 78
  source 1..399: mol_type = other DNA
cctacttcaagttctacaaagaaaacacagctacaactggagcatttactgctggatttacagatgattttgaatggaattaataattacaagaatcccgaactcaccgcgatgctcacaaagaagttttacatgcccaagaaggccacagaactgaaacatcttcagtgtctagaagaagaactcaaacctctggaggaagtgctaaatttagctcaaagcaaaaactttcacttcgaacccagggacgtagtcagcaatatcaacgtatttgttctggaactaaagggatctgaaacaacattcatgtgtgaatatgctgatgagacagcaaccattgtagaatttctgaacagatggattacctttagtcaaagcatcatctcaacactgacttga

SEQ ID NO: 185 - DNA, 399 bp, synthetic construct
  misc_feature 1..399: note = IL-2 analog 79
  source 1..399: mol_type = other DNA
cctacttcaagttctacaaagaaaacacagctacaactggagcatttactgctggatttacagatgattttgaatggaattaataattacaagaatcccgaactcaccgcgatgctcacaaagaagttttacatgcccaagaaggccacagaactgaaacatcttcagtgtctagaagaagaactcaaacctctggaggaagtgctaaatttagctcacagcaaaaactttcacttcgaacccagggacgtagtcagcaatatcaacgtatttgttctggaactaaagggatctgaaacaacattcatgtgtgaatatgctgatgagacagcaaccattgtagaatttctgaacagatggattacctttagtcaaagcatcatctcaacactgacttga

SEQ ID NO: 186 - DNA, 399 bp, synthetic construct
  misc_feature 1..399: note = IL-2 analog 80
  source 1..399: mol_type = other DNA
cctacttcaagttctacaaagaaaacacagctacaactggagcatttactgctggatttacagatgattttgaatggaattaataattacaagaatcccgaactcaccgcgatgctcacaaagaagttttacatgcccaagaaggccacagaactgaaacatcttcagtgtctagaagaagaactcaaacctctggaggaagtgctaaatttagctcacagcaaaaactttcacttcgaaggcagggacgtagtcagcaatatcaacgtatttgttctggaactaaagggatctgaaacaacattcatgtgtgaatatgctgatgagacagcaaccattgtagaatttctgaacagatggattacctttagtcaaagcatcatctcaacactgacttga

SEQ ID NO: 187 - DNA, 399 bp, synthetic construct
  misc_feature 1..399: note = IL-2 analog 81
  source 1..399: mol_type = other DNA
cctacttcaagttctacaaagaaaacacagctacaactggagcatttactgctggatttacagatgattttgaatggaattaataattacaagaatcccgaactcaccgcgatgctcacaaagaagttttacatgcccaagaaggccacagaactgaaacatcttcagtgtctagaagaagaactcaaacctctggaggaagtgctaaatttagctcacagcaaaaactttcacttcgaagtcagggacgtagtcagcaatatcaacgtatttgttctggaactaaagggatctgaaacaacattcatgtgtgaatatgctgatgagacagcaaccattgtagaatttctgaacagatggattacctttagtcaaagcatcatctcaacactgacttga

SEQ ID NO: 188 - DNA, 399 bp, synthetic construct
  misc_feature 1..399: note = IL-2 analog 82
  source 1..399: mol_type = other DNA
cctacttcaagttctacaaagaaaacacagctacaactggagcatttacgtctggatttagaaatgattttgaatggaattaataattacaagaatcccaaactcaccaggatgctcacatttaagttttacatgcccaagaaggccacagaactgaaacatcttcagtgtctagaagaagaactcaaacctctggaggaagtgctaaatttagctcaaagcaaaaactttcactttgaccccagggacgaagtgagcaatatcaacgtatttgttctggaactaaagggatctgaaacaacattcatgtgtgaatatgctgatgagacagcaaccattgtagaatttctgaacagatggattacctttagtcaaagcatcatctcaacactgacttga

SEQ ID NO: 189 - DNA, 399 bp, synthetic construct
  misc_feature 1..399: note = IL-2 analog 83
  source 1..399: mol_type = other DNA
cctacttcaagttctacaaagaaaacacagctacaactggagcatttacgtcgtgatttagaaatgattttgaatggaattaataattacaagaatcccaaactcaccaggatgctcacatttaagttttacatgcccaagaaggccacagaactgaaacatcttcagtgtctagaagaagaactcaaacctctggaggaagtgctaaatttagctcaaagcaaaaactttcactttgaccccagggacgaagtgagcaatatcaacgtatttgttctggaactaaagggatctgaaacaacattcatgtgtgaatatgctgatgagacagcaaccattgtagaatttctgaacagatggattacctttagtcaaagcatcatctcaacactgacttga

SEQ ID NO: 190 - DNA, 399 bp, synthetic construct
  misc_feature 1..399: note = IL-2 analog 84
  source 1..399: mol_type = other DNA
cctacttcaagttctacaaagaaaacacagctacaactggagcatttacgtctggatttagaaatgattttgaatggaattaataattacaagaatcccaaactcaccaggatgctcacatttaagttttacatgcccaagaaggccacagaactgaaacatcttcagtgtctagaagaagaactcaaacctctggaggaagtgctaaatttagctcaaagcaaaaactttcacgtggatcccagggacgaagtgagcaatatcaacgtatttgttctggaactaaagggatctgaaacaacattcatgtgtgaatatgctgatgagacagcaaccattgtagaatttctgaacagatggattacctttagtcaaagcatcatctcaacactgacttga

SEQ ID NO: 191 - DNA, 399 bp, synthetic construct
  misc_feature 1..399: note = IL-2 analog 85
  source 1..399: mol_type = other DNA
cctacttcaagttctacaaagaaaacacagctacaactggagcatttactgctggatttacagatgattttgaatggaattaataattacaagaatcccaaactcaccaggatgctcacatttaagttttacatgcccaagaaggccacagaactgaaacatcttcagtgtctagaagaagaactcaaacctctggaggaagtgctaaatttagctcaaagcaaaaactttcacttcgaacccagggacgtagtcagcaatatcaacgtatttgttctggaactaaagggatctgaaacaacattcatgtgtgaatatgctgatgagacagcaaccattgtagaatttctgaacagatggattacctttagtcaaagcatcatctcaacactgacttga

SEQ ID NO: 192 - DNA, 399 bp, synthetic construct
  misc_feature 1..399: note = IL-2 analog 86
  source 1..399: mol_type = other DNA
cctacttcaagttctacaaagaaaacacagctacaactggagcatttacgtctggatttagaaatgattttgaatggaattaataattacaagaatcccaaactcaccaggatgctcacatttaagttttacatgcccaagaaggccacagaactgaaacatcttcagtgtctagaagaagaactcaaacctctggaggaagtgctaaatttagctcaaagcaaaaactttcacttcgaacccagggacgtagtcagcaatatcaacgtatttgttctggaactaaagggatctgaaacaacattcatgtgtgaatatgctgatgagacagcaaccattgtagaatttctgaacagatggattacctttagtcaaagcatcatctcaacactgacttga

SEQ ID NO: 193 - DNA, 399 bp, synthetic construct
  misc_feature 1..399: note = IL-2 analog 87
  source 1..399: mol_type = other DNA
cctacttcaagttctacaaagaaaacacagctacaactggagcatttacgtcgtgatttagaaatgattttgaatggaattaataattacaagaatcccaaactcaccaggatgctcacatttaagttttacatgcccaagaaggccacagaactgaaacatcttcagtgtctagaagaagaactcaaacctctggaggaagtgctaaatttagctcaaagcaaaaactttcacttcgaacccagggacgtagtcagcaatatcaacgtatttgttctggaactaaagggatctgaaacaacattcatgtgtgaatatgctgatgagacagcaaccattgtagaatttctgaacagatggattacctttagtcaaagcatcatctcaacactgacttga

SEQ ID NO: 194 - DNA, 399 bp, synthetic construct
  misc_feature 1..399: note = IL-2 analog 88
  source 1..399: mol_type = other DNA
cctacttcaagttctacaaagaaaacacagctacaactggagcatttactgctggatttacagatgattttgaatggaattaataattacaagaatcccaaactcaccaggatgctcacatttaagttttacatgcccaagaaggccacagaactgaaacatcttcagtgtctagaagacgaactcaaacctctggaggaagtgctaaatttagctcaaagcaaaaactttcacttcgaacccagggacgtagtcagcaatatcaacgtatttgttctggaactaaagggatctgaaacaacattcatgtgtgaatatgctgatgagacagcaaccattgtagaatttctgaacagatggattacctttagtcaaagcatcatctcaacactgacttga

SEQ ID NO: 195 - DNA, 399 bp, synthetic construct
  misc_feature 1..399: note = IL-2 analog 89
  source 1..399: mol_type = other DNA
cctacttcaagttctacaaagaaaacacagctacaactggagcatttactgctggatttacagatgattttgaatggaattaataattacaagaatcccaaactcaccgcgatgctcacatttaagttttacatgcccaagaaggccacagaactgaaacatcttcagtgtctagaagaagaactcaaacctctggagcaggtgctaaatttagctcaaagcaaaaactttcacttcgaacccagggacgtagtcagcaatatcaacgtatttgttctggaactaaagggatctgaaacaacattcatgtgtgaatatgctgatgagacagcaaccattgtagaatttctgaacagatggattacctttagtcaaagcatcatctcaacactgacttga

SEQ ID NO: 196 - DNA, 399 bp, synthetic construct
  misc_feature 1..399: note = IL-2 analog 90
  source 1..399: mol_type = other DNA
cctacttcaagttctacaaagaaaacacagctacaactggagcatttactgctggatttacagatgattttgaatggaattaataattacaagaatcccaaactcaccaggatgctcacatggaagttttacatgcccaagaaggccacagaactgaaacatcttcagtgtctagaagaagaactcaaacctctggaggaagtgctaaatttagctcaaagcaaaaactttcacttcgaacccagggacgtagtcagcaatatcaacgtatttgttctggaactaaagggatctgaaacaacattcatgtgtgaatatgctgatgagacagcaaccattgtagaatttctgaacagatggattacctttagtcaaagcatcatctcaacactgacttga

SEQ ID NO: 197 - DNA, 399 bp, synthetic construct
  misc_feature 1..399: note = IL-2 analog 91
  source 1..399: mol_type = other DNA
cctacttcaagttctacaaagaaaacacagctacaactggagcatttactgctggatttacagatgattttgaatggaattaataattacaagaatcccaaactcaccaggatgctcacatttaagttttacatgcccaagaaggccacagaactgaaacatcttcagtgtctagaacaagaactcaaacctctggaggaagtgctaaatttagctcaaagcaaaaactttcacttcgaacccagggacgtagtcagcaatatcaacgtatttgttctggaactaaagggatctgaaacaacattcatgtgtgaatatgctgatgagacagcaaccattgtagaatttctgaacagatggattacctttagtcaaagcatcatctcaacactgacttga

SEQ ID NO: 198 - DNA, 399 bp, synthetic construct
  misc_feature 1..399: note = IL-2 analog 92
  source 1..399: mol_type = other DNA
cctacttcaagttctacaaagaaaacacagctacaactggagcatttactgctggatttacagatgattttgaatggaattaataattacaagaatcccaaactcaccaggatgctcacatttaagttttacatgcccaagaaggccacagaactgaaacatcttcagtgtctagaagaagaactcaaacctctggaggaagtgctaaatttagctcaaagcaaaaactttcacttcgaacccagggacgtagtcagcaatatcaacacatttgttctggaactaaagggatctgaaacaacattcatgtgtgaatatgctgatgagacagcaaccattgtagaatttctgaacagatggattacctttagtcaaagcatcatctcaacactgacttga

SEQ ID NO: 199 - DNA, 399 bp, synthetic construct
  misc_feature 1..399: note = IL-2 analog 93
  source 1..399: mol_type = other DNA
cctacttcaagttctacaaagaaaacacagctacaactggagcatttactgctggatttacagatgattttgaatggaattaataattacaagaatcccaaactcaccaggatgctcacatttaagttttacatgcccaagaaggccacagaactgaaacatcttcagtgtctagaagaagaactcaaacctctggaggaagtgctaaatttagctcaaagcaaaaactttcacttcgaacccagggaggtagtcagcaatatcaacacatttgttctggaactaaagggatctgaaacaacattcatgtgtgaatatgctgatgagacagcaaccattgtagaatttctgaacagatggattacctttagtcaaagcatcatctcaacactgacttga

SEQ ID NO: 200 - DNA, 399 bp, synthetic construct
  misc_feature 1..399: note = IL-2 analog 94
  source 1..399: mol_type = other DNA
cctacttcaagttctacaaagaaaacacagctacaactggagcatttactgctggatttacagatgattttgaatggaattaataattacaagaatcccaaactcaccaggatgctcacatttaagttttacatgcccaagaaggccacagaactgaaacatcttcagtgtctagaagaagaactcaaacctctggaggaagtgctaaatttagctcaaagcaaaaactttcacttcgaacccagggacgtagtcagcaatatcaacgtatttgttttcgaattcaagggatctgaaacaacattcatgtgtgaatatgctgatgagacagcaaccattgtagaatttctgaacagatggattacctttagtcaaagcatcatctcaacactgacttga

SEQ ID NO: 201 - DNA, 399 bp, synthetic construct
  misc_feature 1..399: note = IL-2 analog 95
  source 1..399: mol_type = other DNA
cctacttcaagttctacaaagaaaacacagctacaactggagcatttactgctggatttacagatgattttgaatggaattaataattacaagaatcccaaactcaccaggatgctcacatttaagttttacatgcccaagaaggccacagaactgaaacatcttcagtgtctagaagaagaactcaaacctctggaggaagggctaaatttagctcaaagcaaaaactttcacttcgaacccagggacgtagtcagcaatatcaacgtatttgttctggaactaaagggatctgaaacaacattcatgtgtgaatatgctgatgagacagcaaccattgtagaatttctgaacagatggattacctttagtcaaagcatcatctcaacactgacttga

SEQ ID NO: 202 - DNA, 399 bp, synthetic construct
  misc_feature 1..399: note = IL-2 analog 96
  source 1..399: mol_type = other DNA
cctacttcaagttctacaaagaaaacacagctacaactggagcatttactgctggatttacagatgattttgaatggaattaataattacaagaatcccaaactcaccaggatgctcacatttaagttttacatgcccaagaaggccacagaactgaaacatcttcagtgtctagaagaagaactcaaacctctggaggaagggctaaatttagctgcaagcaaaaactttcacttcgaacccagggacgtagtcagcaatatcaacgtatttgttctggaactaaagggatctgaaacaacattcatgtgtgaatatgctgatgagacagcaaccattgtagaatttctgaacagatggattacctttagtcaaagcatcatctcaacactgacttga

SEQ ID NO: 203 - DNA, 399 bp, synthetic construct
  misc_feature 1..399: note = IL-2 analog 97
  source 1..399: mol_type = other DNA
cctacttcaagttctacaaagaaaacacagctacaactggagcatttactgctggatttacagatgattttgaatggaattaataattacaagaatcccaaactcaccgcgatgctcacatttaagttttacatgcccaagaaggccacagaactgaaacatcttcagtgtctagaagaagaactcaaacctctggaggaagtgctaaatttagctcaaagcaaaaactttcactttgaccccagggacttaatcagcaatatcaacgtatttgttctggaactaaagggatctgaaacaacattcatgtgtgaatatgctgatgagacagcaaccattgtagaatttctgaacagatggattacctttagtcaaagcatcatctcaacactgacttga

SEQ ID NO: 204 - DNA, 399 bp, synthetic construct
  misc_feature 1..399: note = IL-2 analog 98
  source 1..399: mol_type = other DNA
cctacttcaagttctacaaagaaaacacagctacaactggagcatttactgctggatttacagatgattttgaatggaattaataattacaagaatcccaaactcaccgcgatgctcacatttaagttttacatgcccaagaaggccacagaactgaaacatcttcagtgtctagaagaagaactcaaacctctggaggaagtgctaaatttagctcaaagcaaaaactttcactttgagcccagggacgtaatcagcaatatcaacgtatttgttctggaactaaagggatctgaaacaacattcatgtgtgaatatgctgatgagacagcaaccattgtagaatttctgaacagatggattacctttagtcaaagcatcatctcaacactgacttga

SEQ ID NO: 205 - DNA, 399 bp, synthetic construct
  misc_feature 1..399: note = IL-2 analog 99
  source 1..399: mol_type = other DNA
cctacttcaagttctacaaagaaaacacagctacaactggagcatttactgctggatttacagatgattttgaatggaattaataattacaagaatcccaaactcaccgcgatgctcacatttaagttttacatgcccaagaaggccacagaactgaaacatcttcagtgtctagaagaagaactcaaacctctggaggaagtgctaaatttagctcaaagcaaaaactttcactttgagcccagggacttagtcagcaatatcaacgtatttgttctggaactaaagggatctgaaacaacattcatgtgtgaatatgctgatgagacagcaaccattgtagaatttctgaacagatggattacctttagtcaaagcatcatctcaacactgacttga

SEQ ID NO: 206 - DNA, 399 bp, synthetic construct
  misc_feature 1..399: note = IL-2 analog 100
  source 1..399: mol_type = other DNA
cctacttcaagttctacaaagaaaacacagctacaactggagcatttactgctggatttacagatgattttgaatggaattaataattacaagaatcccaaactcaccaggatgctcacatttaagttttacatgcccaagaaggccacagaactgaaacatcttcagtgtctagaagaagaactcaaacctctggaggaagtgctaaatttagctcaaagcaaaaactttcacttcgaacccagggactacgtcagcaatatcaacgtatttgttctggaactaaagggatctgaaacaacattcatgtgtgaatatgctgatgagacagcaaccattgtagaatttctgaacagatggattacctttagtcaaagcatcatctcaacactgacttga

SEQ ID NO: 207 - DNA, 399 bp, synthetic construct
  misc_feature 1..399: note = IL-2 analog 101
  source 1..399: mol_type = other DNA
cctacttcaagttctacaaagaaaacacagctacaactggagcatttactgctggatttacagatgattttgaatggaattaataattacaagaatcccaaactcaccaggatgctcacatttaagttttacatgcccaagaaggccacagaactgaaacatcttcagtgtctagaagaagaactcaaacctctggaggaagtgctaaatttagctcaaagcaaaaactttcacttcgaacccagggacctggccagcaatatcaacgtatttgttctggaactaaagggatctgaaacaacattcatgtgtgaatatgctgatgagacagcaaccattgtagaatttctgaacagatggattacctttagtcaaagcatcatctcaacactgacttga

SEQ ID NO: 208 - DNA, 399 bp, synthetic construct
  misc_feature 1..399: note = IL-2 analog 102
  source 1..399: mol_type = other DNA
cctacttcaagttctacaaagaaaacacagctacaactggagcatttactgctggatttacagatgattttgaatggaattaataattacaagaatcccaaactcaccaggatgctcacatttaagttttacatgcccaagaaggccacagaactgaaacatcttcagtgtctagaagaagaactcaaacctctggaggaagtgctaaatttagctcaaagcaaaaactttcacttcgaacccagggacgtagtcagcaatatcaacgtaattgttctggaactaaagggatctgaaacaacattcatgtgtgaatatgctgatgagacagcaaccattgtagaatttctgaacagatggattacctttagtcaaagcatcatctcaacactgacttga

SEQ ID NO: 209 - DNA, 399 bp, synthetic construct
  misc_feature 1..399: note = IL-2 analog 103
  source 1..399: mol_type = other DNA
cctacttcaagttctacaaagaaaacacagctacaactggagcatttacgtctggatttagaaatgattttgaatggaattaataattacaagaatcccaaactcaccgcgatgctcacatttaagttttacatgcccaagaaggccacagaactgaaacatcttcagtgtctagaagaagaactcaaacctctggaggaagtgctaaatttagctcaaagcaaaaactttcacttcgaacccagggacgtagtcagcaatatcaacgtatttgttctggaactaaagggatctgaaacaacattcatgtgtgaatatgctgatgagacagcaaccattgtagaatttctgaacagatggattacctttagtcaaagcatcatctcaacactgacttga

SEQ ID NO: 210 - DNA, 399 bp, synthetic construct
  misc_feature 1..399: note = IL-2 analog 104
  source 1..399: mol_type = other DNA
cctacttcaagttctacaaagaaaacacagctacaactggagcatttacgtctggatttagaaatgattttgaatggaattaataattacaagaatcccaaactcaccaggatgctcacatttaagttttacatgcccaagaaggccacagaactgaaacatcttcagtgtctagaagacgaactcaaacctctggaggaagtgctaaatttagctcaaagcaaaaactttcacttcgaacccagggacgtagtcagcaatatcaacgtatttgttctggaactaaagggatctgaaacaacattcatgtgtgaatatgctgatgagacagcaaccattgtagaatttctgaacagatggattacctttagtcaaagcatcatctcaacactgacttga

SEQ ID NO: 211 - DNA, 399 bp, synthetic construct
  misc_feature 1..399: note = IL-2 analog 105
  source 1..399: mol_type = other DNA
cctacttcaagttctacaaagaaaacacagctacaactggagcatttacgtctggatttagaaatgattttgaatggaattaataattacaagaatcccaaactcaccaggatgctcacatttaagttttacatgcccaagaaggccacagaactgaaacatcttcagtgtctagaagaagaactcaaacctctggaggacgtgctaaatttagctcaaagcaaaaactttcacttcgaacccagggacgtagtcagcaatatcaacgtatttgttctggaactaaagggatctgaaacaacattcatgtgtgaatatgctgatgagacagcaaccattgtagaatttctgaacagatggattacctttagtcaaagcatcatctcaacactgacttga

SEQ ID NO: 212 - protein, 133 aa, synthetic construct
  REGION 1..133: note = General Formula 1
  SITE 1: note = MISC_FEATURE - Xaa is absent
  SITE 18: note = MISC_FEATURE - Xaa is leucine (L) or arginine (R)
  SITE 19: note = MISC_FEATURE - Xaa is leucine (L) or tyrosine (Y)
  SITE 22: note = MISC_FEATURE - Xaa is glutamic acid (E) or glutamine (Q)
  SITE 38: note = MISC_FEATURE - Xaa is alanine (A), aspartic acid (D), or arginine (R)
  SITE 42: note = MISC_FEATURE - Xaa is alanine (A), phenylalanine (F), lysine (K), or tryptophan (W)
  SITE 43: note = MISC_FEATURE - Xaa is glutamic acid (E), lysine (K), or glutamine (Q)
  SITE 45: note = MISC_FEATURE - Xaa is alanine (A) or tyrosine (Y)
  SITE 61: note = MISC_FEATURE - Xaa is aspartic acid (D), glutamic acid (E), glutamine (Q), or arginine (R)
  SITE 68: note = MISC_FEATURE - Xaa is aspartic acid (D) or glutamic acid (E)
  SITE 74: note = MISC_FEATURE - Xaa is histidine (H) or glutamine (Q)
  SITE 80: note = MISC_FEATURE - Xaa is phenylalanine (F), leucine (L), valine (V), or tyrosine (Y)
  SITE 81: note = MISC_FEATURE - Xaa is aspartic acid (D), glutamic acid (E), or arginine (R)
  SITE 84: note = MISC_FEATURE - Xaa is aspartic acid (D) or glutamic acid (E)
  SITE 85: note = MISC_FEATURE - Xaa is alanine (A), glutamic acid (E), glycine (G), leucine (L), valine (V), tryptophan (W), or tyrosine (Y)
  SITE 86: note = MISC_FEATURE - Xaa is alanine (A), glycine (G), isoleucine (I), or valine (V)
  SITE 91: note = MISC_FEATURE - Xaa is threonine (T) or valine (V)
  SITE 92: note = MISC_FEATURE - Xaa is phenylalanine (F), isoleucine (I), or tyrosine (Y)
  SITE 94: note = MISC_FEATURE - Xaa is phenylalanine (F) or leucine (L)
  SITE 96: note = MISC_FEATURE - Xaa is phenylalanine (F) or leucine (L)
XPTSSSTKKTQLQLEHLXXDLXMILNGINNYKNPKLTXMLTXXFXMPKKATELKHLQCLEXELKPLEXVLNLAXSKNFHXXPRXXXSNINXXVXEXKGSETTFMCEYADETATIVEFLNRWITFSQSIISTLT

SEQ ID NO: 213 - protein, 133 aa, synthetic construct
  REGION 1..133: note = General Formula 2
  SITE 1: note = MISC_FEATURE - Xaa is absent
  SITE 18: note = MISC_FEATURE - Xaa is leucine (L) or arginine (R)
  SITE 22: note = MISC_FEATURE - Xaa is glutamic acid (E) or glutamine (Q)
  SITE 38: note = MISC_FEATURE - Xaa is alanine (A) or arginine (R)
  SITE 42: note = MISC_FEATURE - Xaa is phenylalanine (F) or lysine (K)
  SITE 61: note = MISC_FEATURE - Xaa is aspartic acid (D) or glutamic acid (E)
  SITE 68: note = MISC_FEATURE - Xaa is aspartic acid (D) or glutamic acid (E)
  SITE 81: note = MISC_FEATURE - Xaais aspartic acid (D) or glutamic acid (E)
  SITE 85: note = MISC_FEATURE - Xaa is leucine (L) or valine (V)
  SITE 86: note = MISC_FEATURE - Xaa is isoleucine (I) or valine (V)
XPTSSSTKKTQLQLEHLXLDLXMILNGINNYKNPKLTXMLTXKFYMPKKATELKHLQCLEXELKPLEXVLNLAQSKNFHFXPRDXXSNINVFVLELKGSETTFMCEYADETATIVEFLNRWITFSQSIISTLT

SEQ ID NO: 214 - DNA, 33 bp, synthetic construct
  misc_feature 1..33: note = primer #1 (IL2_L12F_F)
  source 1..33: mol_type = other DNA
caaagaaaacacagtttcaactggagcatttac

SEQ ID NO: 215 - DNA, 33 bp, synthetic construct
  misc_feature 1..33: note = primer #2 (IL2_L12F_R)
  source 1..33: mol_type = other DNA
gtaaatgctccagttgaaactgtgttttctttg

SEQ ID NO: 216 - DNA, 33 bp, synthetic construct
  misc_feature 1..33: note = primer #3 (IL2_L12V_F)
  source 1..33: mol_type = other DNA
caaagaaaacacaggtacaactggagcatttac

SEQ ID NO: 217 - DNA, 33 bp, synthetic construct
  misc_feature 1..33: note = primer #4 (IL2_L12V_R)
  source 1..33: mol_type = other DNA
gtaaatgctccagttgtacctgtgttttctttg

SEQ ID NO: 218 - DNA, 39 bp, synthetic construct
  misc_feature 1..39: note = primer #5 (IL2_L18R_L19R_Q22E_F)
  source 1..39: mol_type = other DNA
ctggagcatttacgtcgtgatttagaaatgattttgaat

SEQ ID NO: 219 - DNA, 39 bp, synthetic construct
  misc_feature 1..39: note = primer #6 (IL2_L18R_L19R_Q22E_R)
  source 1..39: mol_type = other DNA
attcaaaatcatttctaaatcacgacgtaaatgctccag

SEQ ID NO: 220 - DNA, 39 bp, synthetic construct
  misc_feature 1..39: note = primer #7 (IL2_L18R_Q22E_F)
  source 1..39: mol_type = other DNA
ctggagcatttacgtctggatttagaaatgattttgaat

SEQ ID NO: 221 - DNA, 39 bp, synthetic construct
  misc_feature 1..39: note = primer #8 (IL2_L18R_Q22E_R)
  source 1..39: mol_type = other DNA
attcaaaatcatttctaaatccagacgtaaatgctccag

SEQ ID NO: 222 - DNA, 33 bp, synthetic construct
  misc_feature 1..33: note = primer #9 (IL2_L19F_F)
  source 1..33: mol_type = other DNA
gagcatttactgttcgatttacagatgattttg

SEQ ID NO: 223 - DNA, 33 bp, synthetic construct
  misc_feature 1..33: note = primer #10 (IL2_L19F_R)
  source 1..33: mol_type = other DNA
caaaatcatctgtaaatcgaacagtaaatgctc

SEQ ID NO: 224 - DNA, 33 bp, synthetic construct
  misc_feature 1..33: note = primer #11 (IL2_L19V_F)
  source 1..33: mol_type = other DNA
gagcatttactggtggatttacagatgattttg

SEQ ID NO: 225 - DNA, 33 bp, synthetic construct
  misc_feature 1..33: note = primer #12 (IL2_L19V_R)
  source 1..33: mol_type = other DNA
caaaatcatctgtaaatccaccagtaaatgctc

SEQ ID NO: 226 - DNA, 33 bp, synthetic construct
  misc_feature 1..33: note = primer #13 (IL2_L19Y_F)
  source 1..33: mol_type = other DNA
caactggagcatttactgtacgatttacagatg

SEQ ID NO: 227 - DNA, 33 bp, synthetic construct
  misc_feature 1..33: note = primer #14 (IL2_L19Y_R)
  source 1..33: mol_type = other DNA
catctgtaaatcgtacagtaaatgctccagttg

SEQ ID NO: 228 - DNA, 34 bp, synthetic construct
  misc_feature 1..34: note = primer #15 (IL2_D20F_F)
  source 1..34: mol_type = other DNA
ggagcatttactgctgtttttacagatgattttg

SEQ ID NO: 229 - DNA, 34 bp, synthetic construct
  misc_feature 1..34: note = primer #16 (IL2_D20F_R)
  source 1..34: mol_type = other DNA
caaaatcatctgtaaaaacagcagtaaatgctcc

SEQ ID NO: 230 - DNA, 33 bp, synthetic construct
  misc_feature 1..33: note = primer #17 (IL2_D20V_F)
  source 1..33: mol_type = other DNA
gagcatttactgctggttttacagatgattttg

SEQ ID NO: 231 - DNA, 33 bp, synthetic construct
  misc_feature 1..33: note = primer #18 (IL2_D20V_R)
  source 1..33: mol_type = other DNA
caaaatcatctgtaaaaccagcagtaaatgctc

SEQ ID NO: 232 - DNA, 33 bp, synthetic construct
  misc_feature 1..33: note = primer #19 (IL2_K32C_F)
  source 1..33: mol_type = other DNA
ggaattaataattactgtaatcccaaactcacc

SEQ ID NO: 233 - DNA, 33 bp, synthetic construct
  misc_feature 1..33: note = primer #20 (IL2_K32C_R)
  source 1..33: mol_type = other DNA
ggtgagtttgggattacagtaattattaattcc

SEQ ID NO: 234 - DNA, 33 bp, synthetic construct
  misc_feature 1..33: note = primer #21 (IL2_K35C_F)
  source 1..33: mol_type = other DNA
aattacaagaatccctgtctcaccaggatgctc

SEQ ID NO: 235 - DNA, 33 bp, synthetic construct
  misc_feature 1..33: note = primer #22 (IL2_K35C_R)
  source 1..33: mol_type = other DNA
gagcatcctggtgagacagggattcttgtaatt

SEQ ID NO: 236 - DNA, 33 bp, synthetic construct
  misc_feature 1..33: note = primer #23 (IL2_K35E_F)
  source 1..33: mol_type = other DNA
taattacaagaatcccgaactcaccgcgatgct

SEQ ID NO: 237 - DNA, 33 bp, synthetic construct
  misc_feature 1..33: note = primer #24 (IL2_K35E_R)
  source 1..33: mol_type = other DNA
agcatcgcggtgagttcgggattcttgtaatta

SEQ ID NO: 238 - DNA, 25 bp, synthetic construct
  misc_feature 1..25: note = primer #25 (IL2_R38A_F)
  source 1..25: mol_type = other DNA
ccaaactcaccgcgatgctcacatt

SEQ ID NO: 239 - DNA, 25 bp, synthetic construct
  misc_feature 1..25: note = primer #26 (IL2_R38A_R)
  source 1..25: mol_type = other DNA
aatgtgagcatcgcggtgagtttgg

SEQ ID NO: 240 - DNA, 33 bp, synthetic construct
  misc_feature 1..33: note = primer #27 (IL2_R38A_F42F_F)
  source 1..33: mol_type = other DNA
caccgcgatgctcacatttaagttttacatgcc

SEQ ID NO: 241 - DNA, 33 bp, synthetic construct
  misc_feature 1..33: note = primer #28 (IL2_R38A_F42F_R)
  source 1..33: mol_type = other DNA
ggcatgtaaaacttaaatgtgagcatcgcggtg

SEQ ID NO: 242 - DNA, 25 bp, synthetic construct
  misc_feature 1..25: note = primer #29 (IL2_A38R_F)
  source 1..25: mol_type = other DNA
ccaaactcaccaggatgctcacatt

SEQ ID NO: 243 - DNA, 25 bp, synthetic construct
  misc_feature 1..25: note = primer #30 (IL2_A38R_R)
  source 1..25: mol_type = other DNA
aatgtgagcatcctggtgagtttgg

SEQ ID NO: 244 - DNA, 30 bp, synthetic construct
  misc_feature 1..30: note = primer #31 (IL2_R38D_F)
  source 1..30: mol_type = other DNA
aagaatcccaaactcaccgatatgctcaca

SEQ ID NO: 245 - DNA, 30 bp, synthetic construct
  misc_feature 1..30: note = primer #32 (IL2_R38D_R)
  source 1..30: mol_type = other DNA
tgtgagcatatcggtgagtttgggattctt

SEQ ID NO: 246 - DNA, 30 bp, synthetic construct
  misc_feature 1..30: note = primer #33 (IL2_F42A_F)
  source 1..30: mol_type = other DNA
ccaggatgctcacagctaagttttacatgc

SEQ ID NO: 247 - DNA, 30 bp, synthetic construct
  misc_feature 1..30: note = primer #34 (IL2_F42A_R)
  source 1..30: mol_type = other DNA
gcatgtaaaacttagctgtgagcatcctgg

SEQ ID NO: 248 - DNA, 30 bp, synthetic construct
  misc_feature 1..30: note = primer #35 (IL2_F42K_F)
  source 1..30: mol_type = other DNA
ccaggatgctcacaaagaagttttacatgc

SEQ ID NO: 249 - DNA, 30 bp, synthetic construct
  misc_feature 1..30: note = primer #36 (IL2_F42K_R)
  source 1..30: mol_type = other DNA
gcatgtaaaacttctttgtgagcatcctgg

SEQ ID NO: 250 - DNA, 30 bp, synthetic construct
  misc_feature 1..30: note = primer #37 (IL2_F42K_K43E_F)
  source 1..30: mol_type = other DNA
atgctcacaaaggagttttacatgcccaag

SEQ ID NO: 251 - DNA, 30 bp, synthetic construct
  misc_feature 1..30: note = primer #38 (IL2_F42K_K43E_R)
  source 1..30: mol_type = other DNA
cttgggcatgtaaaactcctttgtgagcat

SEQ ID NO: 252 - DNA, 30 bp, synthetic construct
  misc_feature 1..30: note = primer #39 (IL2_F42K_K43Q_F)
  source 1..30: mol_type = other DNA
atgctcacaaagcagttttacatgcccaag

SEQ ID NO: 253 - DNA, 30 bp, synthetic construct
  misc_feature 1..30: note = primer #40 (IL2_F42K_K43Q_R)
  source 1..30: mol_type = other DNA
cttgggcatgtaaaactgctttgtgagcat

SEQ ID NO: 254 - DNA, 30 bp, synthetic construct
  misc_feature 1..30: note = primer #41 (IL2_K42F_F)
  source 1..30: mol_type = other DNA
ccaggatgctcacatttaagttttacatgc

SEQ ID NO: 255 - DNA, 30 bp, synthetic construct
  misc_feature 1..30: note = primer #42 (IL2_K42F_R)
  source 1..30: mol_type = other DNA
gcatgtaaaacttaaatgtgagcatcctgg

SEQ ID NO: 256 - DNA, 39 bp, synthetic construct
  misc_feature 1..39: note = primer #43 (IL2_K42F_F_long)
  source 1..39: mol_type = other DNA
ctcaccaggatgctcacatttaagttttacatgcccaag

SEQ ID NO: 257 - DNA, 39 bp, synthetic construct
  misc_feature 1..39: note = primer #44 (IL2_K42F_R_long)
  source 1..39: mol_type = other DNA
cttgggcatgtaaaacttaaatgtgagcatcctggtgag

SEQ ID NO: 258 - DNA, 33 bp, synthetic construct
  misc_feature 1..33: note = primer #45 (IL2_F42W_F)
  source 1..33: mol_type = other DNA
accaggatgctcacatggaagttttacatgccc

SEQ ID NO: 259 - DNA, 33 bp, synthetic construct
  misc_feature 1..33: note = primer #46 (IL2_F42W_R)
  source 1..33: mol_type = other DNA
gggcatgtaaaacttccatgtgagcatcctggt

SEQ ID NO: 260 - DNA, 33 bp, synthetic construct
  misc_feature 1..33: note = primer #47 (IL2_K43C_F)
  source 1..33: mol_type = other DNA
aggatgctcacattttgtttttacatgcccaag

SEQ ID NO: 261 - DNA, 33 bp, synthetic construct
  misc_feature 1..33: note = primer #48 (IL2_K43C_R)
  source 1..33: mol_type = other DNA
cttgggcatgtaaaaacaaaatgtgagcatcct

SEQ ID NO: 262 - DNA, 19 bp, synthetic construct
  misc_feature 1..19: note = primer #49 (IL2_Y45A_F)
  source 1..19: mol_type = other DNA
gaagtttgccatgcccaag

SEQ ID NO: 263 - DNA, 19 bp, synthetic construct
  misc_feature 1..19: note = primer #50 (IL2_Y45A_R)
  source 1..19: mol_type = other DNA
cttgggcatggcaaacttc

SEQ ID NO: 264 - DNA, 34 bp, synthetic construct
  misc_feature 1..34: note = primer #51 (IL2_Y45A_F_long)
  source 1..34: mol_type = other DNA
gctcacaaagaagtttgccatgcccaagaaggcc

SEQ ID NO: 265 - DNA, 34 bp, synthetic construct
  misc_feature 1..34: note = primer #52 (IL2_Y45A_R_long)
  source 1..34: mol_type = other DNA
ggccttcttgggcatggcaaacttctttgtgagc

SEQ ID NO: 266 - DNA, 33 bp, synthetic construct
  misc_feature 1..33: note = primer #53 (IL2_K48C_F)
  source 1..33: mol_type = other DNA
aagttttacatgccctgtaaggccacagaactg

SEQ ID NO: 267 - DNA, 33 bp, synthetic construct
  misc_feature 1..33: note = primer #54 (IL2_K48C_R)
  source 1..33: mol_type = other DNA
cagttctgtggccttacagggcatgtaaaactt

SEQ ID NO: 268 - DNA, 33 bp, synthetic construct
  misc_feature 1..33: note = primer #55 (IL2_K49C_F)
  source 1..33: mol_type = other DNA
ttttacatgcccaagtgtgccacagaactgaaa

SEQ ID NO: 269 - DNA, 33 bp, synthetic construct
  misc_feature 1..33: note = primer #56 (IL2_K49C_R)
  source 1..33: mol_type = other DNA
tttcagttctgtggcacacttgggcatgtaaaa

SEQ ID NO: 270 - DNA, 33 bp, synthetic construct
  misc_feature 1..33: note = primer #57 (IL2_E61D_F)
  source 1..33: mol_type = other DNA
cttcagtgtctagaagacgaactcaaacctctg

SEQ ID NO: 271 - DNA, 33 bp, synthetic construct
  misc_feature 1..33: note = primer #58 (IL2_E61D_R)
  source 1..33: mol_type = other DNA
cagaggtttgagttcgtcttctagacactgaag

SEQ ID NO: 272 - DNA, 33 bp, synthetic construct
  misc_feature 1..33: note = primer #59 (IL2_E61Q_F)
  source 1..33: mol_type = other DNA
cttcagtgtctagaacaagaactcaaacctctg

SEQ ID NO: 273 - DNA, 33 bp, synthetic construct
  misc_feature 1..33: note = primer #60 (IL2_E61Q_R)
  source 1..33: mol_type = other DNA
cagaggtttgagttcttgttctagacactgaag

SEQ ID NO: 274 - DNA, 30 bp, synthetic construct
  misc_feature 1..30: note = primer #61 (IL2_E61R_F)
  source 1..30: mol_type = other DNA
cttcagtgtctagaacgggaactcaaacct

SEQ ID NO: 275 - DNA, 30 bp, synthetic construct
  misc_feature 1..30: note = primer #62 (IL2_E61R_R)
  source 1..30: mol_type = other DNA
aggtttgagttcccgttctagacactgaag

SEQ ID NO: 276 - DNA, 33 bp, synthetic construct
  misc_feature 1..33: note = primer #63 (IL2_E68D_F)
  source 1..33: mol_type = other DNA
ctcaaacctctggaggacgtgctaaatttagct

SEQ ID NO: 277 - DNA, 33 bp, synthetic construct
  misc_feature 1..33: note = primer #64 (IL2_E68D_R)
  source 1..33: mol_type = other DNA
agctaaatttagcacgtcctccagaggtttgag

SEQ ID NO: 278 - DNA, 33 bp, synthetic construct
  misc_feature 1..33: note = primer #65 (IL2_E68Q_F)
  source 1..33: mol_type = other DNA
ctcaaacctctggagcaggtgctaaatttagct

SEQ ID NO: 279 - DNA, 33 bp, synthetic construct
  misc_feature 1..33: note = primer #66 (IL2_E68Q_R)
  source 1..33: mol_type = other DNA
agctaaatttagcacctgctccagaggtttgag

SEQ ID NO: 280 - DNA, 32 bp, synthetic construct
  misc_feature 1..32: note = primer #67 (IL2_V69G_F)
  source 1..32: mol_type = other DNA
caaacctctggaggaagggctaaatttagctc

SEQ ID NO: 281 - DNA, 32 bp, synthetic construct
  misc_feature 1..32: note = primer #68 (IL2_V69G_R)
  source 1..32: mol_type = other DNA
gagctaaatttagcccttcctccagaggtttg

SEQ ID NO: 282 - DNA, 40 bp, synthetic construct
  misc_feature 1..40: note = primer #69 (IL2_V69G_Q74A_F)
  source 1..40: mol_type = other DNA
ctggaggaagggctaaatttagctgcaagcaaaaactttc

SEQ ID NO: 283 - DNA, 40 bp, synthetic construct
  misc_feature 1..40: note = primer #70 (IL2_V69G_Q74A_R)
  source 1..40: mol_type = other DNA
gaaagtttttgcttgcagctaaatttagcccttcctccag

SEQ ID NO: 284 - DNA, 24 bp, synthetic construct
  misc_feature 1..24: note = primer #71 (IL2_Q74H_F)
  source 1..24: mol_type = other DNA
ctaaatttagctcacagcaaaaac

SEQ ID NO: 285 - DNA, 24 bp, synthetic construct
  misc_feature 1..24: note = primer #72 (IL2_Q74H_R)
  source 1..24: mol_type = other DNA
gtttttgctgtgagctaaatttag

SEQ ID NO: 286 - DNA, 33 bp, synthetic construct
  misc_feature 1..33: note = primer #73 (IL2_K76C_F)
  source 1..33: mol_type = other DNA
aatttagctcaaagctgtaactttcacttaaga

SEQ ID NO: 287 - DNA, 33 bp, synthetic construct
  misc_feature 1..33: note = primer #74 (IL2_K76C_R)
  source 1..33: mol_type = other DNA
tcttaagtgaaagttacagctttgagctaaatt

SEQ ID NO: 288 - DNA, 32 bp, synthetic construct
  misc_feature 1..32: note = primer #75 (IL2_L80D_R81E_F)
  source 1..32: mol_type = other DNA
aaagcaaaaactttcacgacgaacccagggac

SEQ ID NO: 289 - DNA, 32 bp, synthetic construct
  misc_feature 1..32: note = primer #76 (IL2_L80D_R81E_R)
  source 1..32: mol_type = other DNA
gtccctgggttcgtcgtgaaagtttttgcttt

SEQ ID NO: 290 - DNA, 29 bp, synthetic construct
  misc_feature 1..29: note = primer #77 (IL2_L80F_F)
  source 1..29: mol_type = other DNA
gcaaaaactttcactttagacccagggac

SEQ ID NO: 291 - DNA, 29 bp, synthetic construct
  misc_feature 1..29: note = primer #78 (IL2_L80F_R)
  source 1..29: mol_type = other DNA
gtccctgggtctaaagtgaaagtttttgc

SEQ ID NO: 292 - DNA, 29 bp, synthetic construct
  misc_feature 1..29: note = primer #79 (IL2_L80F_R81D_F)
  source 1..29: mol_type = other DNA
gcaaaaactttcactttgaccccagggac

SEQ ID NO: 293 - DNA, 29 bp, synthetic construct
  misc_feature 1..29: note = primer #80 (IL2_L80F_R81D_R)
  source 1..29: mol_type = other DNA
gtccctggggtcaaagtgaaagtttttgc

SEQ ID NO: 294 - DNA, 32 bp, synthetic construct
  misc_feature 1..32: note = primer #81 (IL2_L80F_R81E_F)
  source 1..32: mol_type = other DNA
aaagcaaaaactttcacttcgaacccagggac

SEQ ID NO: 295 - DNA, 32 bp, synthetic construct
  misc_feature 1..32: note = primer #82 (IL2_L80F_R81E_R)
  source 1..32: mol_type = other DNA
gtccctgggttcgaagtgaaagtttttgcttt

SEQ ID NO: 296 - DNA, 32 bp, synthetic construct
  misc_feature 1..32: note = primer #83 (IL2_L80V_R81D_F)
  source 1..32: mol_type = other DNA
aaagcaaaaactttcacgtggatcccagggac

SEQ ID NO: 297 - DNA, 32 bp, synthetic construct
  misc_feature 1..32: note = primer #84 (IL2_L80V_R81D_R)
  source 1..32: mol_type = other DNA
gtccctgggatccacgtgaaagtttttgcttt

SEQ ID NO: 298 - DNA, 32 bp, synthetic construct
  misc_feature 1..32: note = primer #85 (IL2_L80W_R81E_F)
  source 1..32: mol_type = other DNA
aaagcaaaaactttcactgggaacccagggac

SEQ ID NO: 299 - DNA, 32 bp, synthetic construct
  misc_feature 1..32: note = primer #86 (IL2_L80W_R81E_R)
  source 1..32: mol_type = other DNA
gtccctgggttcccagtgaaagtttttgcttt

SEQ ID NO: 300 - DNA, 29 bp, synthetic construct
  misc_feature 1..29: note = primer #87 (IL2_L80Y_R81D_F)
  source 1..29: mol_type = other DNA
gcaaaaactttcactatgaccccagggac

SEQ ID NO: 301 - DNA, 29 bp, synthetic construct
  misc_feature 1..29: note = primer #88 (IL2_L80Y_R81D_R)
  source 1..29: mol_type = other DNA
gtccctggggtcatagtgaaagtttttgc

SEQ ID NO: 302 - DNA, 32 bp, synthetic construct
  misc_feature 1..32: note = primer #89 (IL2_L80Y_R81E_F)
  source 1..32: mol_type = other DNA
aaagcaaaaactttcactacgaacccagggac

SEQ ID NO: 303 - DNA, 32 bp, synthetic construct
  misc_feature 1..32: note = primer #90 (IL2_L80Y_R81E_R)
  source 1..32: mol_type = other DNA
gtccctgggttcgtagtgaaagtttttgcttt

SEQ ID NO: 304 - DNA, 32 bp, synthetic construct
  misc_feature 1..32: note = primer #91 (IL2_L80Y_R81N_F)
  source 1..32: mol_type = other DNA
aaagcaaaaactttcactacaaccccagggac

SEQ ID NO: 305 - DNA, 32 bp, synthetic construct
  misc_feature 1..32: note = primer #92 (IL2_L80Y_R81N_R)
  source 1..32: mol_type = other DNA
gtccctggggttgtagtgaaagtttttgcttt

SEQ ID NO: 306 - DNA, 29 bp, synthetic construct
  misc_feature 1..29: note = primer #93 (IL2_L80Y_R81R_F)
  source 1..29: mol_type = other DNA
gcaaaaactttcactatagacccagggac

SEQ ID NO: 307 - DNA, 29 bp, synthetic construct
  misc_feature 1..29: note = primer #94 (IL2_L80Y_R81R_R)
  source 1..29: mol_type = other DNA
gtccctgggtctatagtgaaagtttttgc

SEQ ID NO: 308 - DNA, 31 bp, synthetic construct
  misc_feature 1..31: note = primer #95 (IL2_R81D_D84E_F)
  source 1..31: mol_type = other DNA
ctttcacttagaccccagggagttaatcagc

SEQ ID NO: 309 - DNA, 31 bp, synthetic construct
  misc_feature 1..31: note = primer #96 (IL2_R81D_D84E_R)
  source 1..31: mol_type = other DNA
gctgattaactccctggggtctaagtgaaag

SEQ ID NO: 310 - DNA, 34 bp, synthetic construct
  misc_feature 1..34: note = primer #97 (IL2_R81D_F)
  source 1..34: mol_type = other DNA
caaaaactttcacttagaccccagggacttaatc

SEQ ID NO: 311 - DNA, 34 bp, synthetic construct
  misc_feature 1..34: note = primer #98 (IL2_R81D_R)
  source 1..34: mol_type = other DNA
gattaagtccctggggtctaagtgaaagtttttg

SEQ ID NO: 312 - DNA, 51 bp, synthetic construct
  misc_feature 1..51: note = primer #99 (IL2_R81D_F_long)
  source 1..51: mol_type = other DNA
ctcaaagcaaaaactttcacttagaccccagggacttaatcagcaaatatc

SEQ ID NO: 313 - DNA, 51 bp, synthetic construct
  misc_feature 1..51: note = primer #100 (IL2_R81D_R_long)
  source 1..51: mol_type = other DNA
gatatttgctgattaagtccctggggtctaagtgaaagtttttgctttgag

SEQ ID NO: 314 - DNA, 43 bp, synthetic construct
  misc_feature 1..43: note = primer #101 (IL2_R81E_D84E_L85V_I86V_V91T_I92F_F)
  source 1..43: mol_type = other DNA
gaacccagggaggtagtcagcaatatcaacacatttgttctgg

SEQ ID NO: 315 - DNA, 43 bp, synthetic construct
  misc_feature 1..43: note = primer #102 (IL2_R81E_D84E_L85V_I86V_V91T_I92F_R)
  source 1..43: mol_type = other DNA
ccagaacaaatgtgttgatattgctgactacctccctgggttc

SEQ ID NO: 316 - DNA, 31 bp, synthetic construct
  misc_feature 1..31: note = primer #103 (IL2_R81E_F)
  source 1..31: mol_type = other DNA
aaactttcacttagaacccagggacttaatc

SEQ ID NO: 317 - DNA, 31 bp, synthetic construct
  misc_feature 1..31: note = primer #104 (IL2_R81E_R)
  source 1..31: mol_type = other DNA
gattaagtccctgggttctaagtgaaagttt

SEQ ID NO: 318 - DNA, 33 bp, synthetic construct
  misc_feature 1..33: note = primer #105 (IL2_P82G_F)
  source 1..33: mol_type = other DNA
aactttcacttcgaaggcagggacgtagtcagc

SEQ ID NO: 319 - DNA, 33 bp, synthetic construct
  misc_feature 1..33: note = primer #106 (IL2_P82G_R)
  source 1..33: mol_type = other DNA
gctgactacgtccctgccttcgaagtgaaagtt

SEQ ID NO: 320 - DNA, 33 bp, synthetic construct
  misc_feature 1..33: note = primer #107 (IL2_P82V_F)
  source 1..33: mol_type = other DNA
aactttcacttcgaagtcagggacgtagtcagc

SEQ ID NO: 321 - DNA, 33 bp, synthetic construct
  misc_feature 1..33: note = primer #108 (IL2_P82V_R)
  source 1..33: mol_type = other DNA
gctgactacgtccctgacttcgaagtgaaagtt

SEQ ID NO: 322 - DNA, 34 bp, synthetic construct
  misc_feature 1..34: note = primer #109 (IL2_D84E_F)
  source 1..34: mol_type = other DNA
cttaagacccagggagttaatcagcaatatcaac

SEQ ID NO: 323 - DNA, 34 bp, synthetic construct
  misc_feature 1..34: note = primer #110 (IL2_D84E_R)
  source 1..34: mol_type = other DNA
gttgatattgctgattaactccctgggtcttaag

SEQ ID NO: 324 - DNA, 32 bp, synthetic construct
  misc_feature 1..32: note = primer #111 (IL2_D84F_F)
  source 1..32: mol_type = other DNA
cacttagaccccaggttcttaatcagcaatat

SEQ ID NO: 325 - DNA, 32 bp, synthetic construct
  misc_feature 1..32: note = primer #112 (IL2_D84F_R)
  source 1..32: mol_type = other DNA
atattgctgattaagaacctggggtctaagtg

SEQ ID NO: 326 - DNA, 31 bp, synthetic construct
  misc_feature 1..31: note = primer #113 (IL2_D84V_F)
  source 1..31: mol_type = other DNA
acttagaccccagggtcttaatcagcaatat

SEQ ID NO: 327 - DNA, 31 bp, synthetic construct
  misc_feature 1..31: note = primer #114 (IL2_D84V_R)
  source 1..31: mol_type = other DNA
atattgctgattaagaccctggggtctaagt

SEQ ID NO: 328 - DNA, 35 bp, synthetic construct
  misc_feature 1..35: note = primer #115 (IL2_L85A_I86A_F)
  source 1..35: mol_type = other DNA
ctttgaccccagggacgctgccagcaatatcaacg

SEQ ID NO: 329 - DNA, 35 bp, synthetic construct
  misc_feature 1..35: note = primer #116 (IL2_L85A_I86A_R)
  source 1..35: mol_type = other DNA
cgttgatattgctggcagcgtccctggggtcaaag

SEQ ID NO: 330 - DNA, 30 bp, synthetic construct
  misc_feature 1..30: note = primer #117 (IL2_L85E_I86V_F)
  source 1..30: mol_type = other DNA
cccagggacgaagtgagcaatatcaacgta

SEQ ID NO: 331 - DNA, 30 bp, synthetic construct
  misc_feature 1..30: note = primer #118 (IL2_L85E_I86V_R)
  source 1..30: mol_type = other DNA
tacgttgatattgctcacttcgtccctggg

SEQ ID NO: 332 - DNA, 27 bp, synthetic construct
  misc_feature 1..27: note = primer #119 (IL2_L85F_I86L_F)
  source 1..27: mol_type = other DNA
cccagggacttcctcagcaatatcaac

SEQ ID NO: 333 - DNA, 27 bp, synthetic construct
  misc_feature 1..27: note = primer #120 (IL2_L85F_I86L_R)
  source 1..27: mol_type = other DNA
gttgatattgctgaggaagtccctggg

SEQ ID NO: 334 - DNA, 27 bp, synthetic construct
  misc_feature 1..27: note = primer #121 (IL2_L85F_I86V_F)
  source 1..27: mol_type = other DNA
cccagggacttcgtcagcaatatcaac

SEQ ID NO: 335 - DNA, 27 bp, synthetic construct
  misc_feature 1..27: note = primer #122 (IL2_L85F_I86V_R)
  source 1..27: mol_type = other DNA
gttgatattgctgacgaagtccctggg

SEQ ID NO: 336 - DNA, 27 bp, synthetic construct
  misc_feature 1..27: note = primer #123 (IL2_L85G_I86A_F)
  source 1..27: mol_type = other DNA
cccagggacggagccagcaatatcaac

SEQ ID NO: 337 - DNA, 27 bp, synthetic construct
  misc_feature 1..27: note = primer #124 (IL2_L85G_I86A_R)
  source 1..27: mol_type = other DNA
gttgatattgctggctccgtccctggg

SEQ ID NO: 338 - DNA, 35 bp, synthetic construct
  misc_feature 1..35: note = primer #125 (IL2_L85G_I86V_F)
  source 1..35: mol_type = other DNA
ctttgaccccagggacggtgttagcaatatcaacg

SEQ ID NO: 339 - DNA, 35 bp, synthetic construct
  misc_feature 1..35: note = primer #126 (IL2_L85G_I86V_R)
  source 1..35: mol_type = other DNA
cgttgatattgctaacccagtccctggggtcaaag

SEQ ID NO: 340 - DNA, 27 bp, synthetic construct
  misc_feature 1..27: note = primer #127 (IL2_L85I_I86V_F)
  source 1..27: mol_type = other DNA
cccagggacatagtcagcaatatcaac

SEQ ID NO: 341 - DNA, 27 bp, synthetic construct
  misc_feature 1..27: note = primer #128 (IL2_L85I_I86V_R)
  source 1..27: mol_type = other DNA
gttgatattgctgactatgtccctggg

SEQ ID NO: 342 - DNA, 34 bp, synthetic construct
  misc_feature 1..34: note = primer #129 (IL2_L85L_I86A_F)
  source 1..34: mol_type = other DNA
cttcgaacccagggacctggccagcaatatcaac

SEQ ID NO: 343 - DNA, 34 bp, synthetic construct
  misc_feature 1..34: note = primer #130 (IL2_L85L_I86A_R)
  source 1..34: mol_type = other DNA
gttgatattgctggccaggtccctgggttcgaag

SEQ ID NO: 344 - DNA, 34 bp, synthetic construct
  misc_feature 1..34: note = primer #131 (IL2_L85L_I86V_F)
  source 1..34: mol_type = other DNA
ctttgagcccagggacttagtcagcaatatcaac

SEQ ID NO: 345 - DNA, 34 bp, synthetic construct
  misc_feature 1..34: note = primer #132 (IL2_L85L_I86V_R)
  source 1..34: mol_type = other DNA
gttgatattgctgactaagtccctgggctcaaag

SEQ ID NO: 346 - DNA, 27 bp, synthetic construct
  misc_feature 1..27: note = primer #133 (IL2_L85T_I86G_F)
  source 1..27: mol_type = other DNA
cccagggacacaggcagcaatatcaac

SEQ ID NO: 347 - DNA, 27 bp, synthetic construct
  misc_feature 1..27: note = primer #134 (IL2_L85T_I86G_R)
  source 1..27: mol_type = other DNA
gttgatattgctgcctgtgtccctggg

SEQ ID NO: 348 - DNA, 29 bp, synthetic construct
  misc_feature 1..29: note = primer #135 (IL2_L85V_I86G_F)
  source 1..29: mol_type = other DNA
cccagggacgtaggcagcaatatcaacgt

SEQ ID NO: 349 - DNA, 29 bp, synthetic construct
  misc_feature 1..29: note = primer #136 (IL2_L85V_I86G_R)
  source 1..29: mol_type = other DNA
acgttgatattgctgcctacgtccctggg

SEQ ID NO: 350 - DNA, 31 bp, synthetic construct
  misc_feature 1..31: note = primer #137 (IL2_L85V_I86I_codon_F)
  source 1..31: mol_type = other DNA
gaacccagggacgtaatcagcaatatcaacg

SEQ ID NO: 351 - DNA, 31 bp, synthetic construct
  misc_feature 1..31: note = primer #138 (IL2_L85V_I86I_codon_R)
  source 1..31: mol_type = other DNA
cgttgatattgctgattacgtccctgggttc

SEQ ID NO: 352 - DNA, 30 bp, synthetic construct
  misc_feature 1..30: note = primer #139 (IL2_L85V_I86V_F)
  source 1..30: mol_type = other DNA
gacccagggacgtagtcagcaatatcaacg

SEQ ID NO: 353 - DNA, 30 bp, synthetic construct
  misc_feature 1..30: note = primer #140 (IL2_L85V_I86V_R)
  source 1..30: mol_type = other DNA
cgttgatattgctgactacgtccctgggtc

SEQ ID NO: 354 - DNA, 29 bp, synthetic construct
  misc_feature 1..29: note = primer #141 (IL2_L85W_I86V_F)
  source 1..29: mol_type = other DNA
cccagggactgggtcagcaatatcaacgt

SEQ ID NO: 355 - DNA, 29 bp, synthetic construct
  misc_feature 1..29: note = primer #142 (IL2_L85W_I86V_R)
  source 1..29: mol_type = other DNA
acgttgatattgctgacccagtccctggg

SEQ ID NO: 356 - DNA, 30 bp, synthetic construct
  misc_feature 1..30: note = primer #143 (IL2_L85W_I86V_Long_F)
  source 1..30: mol_type = other DNA
tttgaccccagggactgggtcagcaatatc

SEQ ID NO: 357 - DNA, 30 bp, synthetic construct
  misc_feature 1..30: note = primer #144 (IL2_L85W_I86V_Long_R)
  source 1..30: mol_type = other DNA
gatattgctgacccagtccctggggtcaaa

SEQ ID NO: 358 - DNA, 34 bp, synthetic construct
  misc_feature 1..34: note = primer #145 (IL2_L85Y_I86V_F)
  source 1..34: mol_type = other DNA
cttcgaacccagggactacgtcagcaatatcaac

SEQ ID NO: 359 - DNA, 34 bp, synthetic construct
  misc_feature 1..34: note = primer #146 (IL2_L85Y_I86V_R)
  source 1..34: mol_type = other DNA
gttgatattgctgacgtagtccctgggttcgaag

SEQ ID NO: 360 - DNA, 31 bp, synthetic construct
  misc_feature 1..31: note = primer #147 (IL2_I86V_V91T_I92F_F)
  source 1..31: mol_type = other DNA
gtcagcaatatcaacacatttgttctggaac

SEQ ID NO: 361 - DNA, 31 bp, synthetic construct
  misc_feature 1..31: note = primer #148 (IL2_I86V_V91T_I92F_R)
  source 1..31: mol_type = other DNA
gttccagaacaaatgtgttgatattgctgac

SEQ ID NO: 362 - DNA, 33 bp, synthetic construct
  misc_feature 1..33: note = primer #149 (IL2_S87C_F)
  source 1..33: mol_type = other DNA
cccagggacttaatctgcaatatcaacgtaata

SEQ ID NO: 363 - DNA, 33 bp, synthetic construct
  misc_feature 1..33: note = primer #150 (IL2_S87C_R)
  source 1..33: mol_type = other DNA
tattacgttgatattgcagattaagtccctggg

SEQ ID NO: 364 - DNA, 34 bp, synthetic construct
  misc_feature 1..34: note = primer #151 (IL2_N88F_F)
  source 1..34: mol_type = other DNA
cagggacttaatcagctttatcaacgtatttgtt

SEQ ID NO: 365 - DNA, 34 bp, synthetic construct
  misc_feature 1..34: note = primer #152 (IL2_N88F_R)
  source 1..34: mol_type = other DNA
aacaaatacgttgataaagctgattaagtccctg

SEQ ID NO: 366 - DNA, 33 bp, synthetic construct
  misc_feature 1..33: note = primer #153 (IL2_N88Q_F)
  source 1..33: mol_type = other DNA
gggacttaatcagccaaatcaacgtaatagttc

SEQ ID NO: 367 - DNA, 33 bp, synthetic construct
  misc_feature 1..33: note = primer #154 (IL2_N88Q_R)
  source 1..33: mol_type = other DNA
gaactattacgttgatttggctgattaagtccc

SEQ ID NO: 368 - DNA, 34 bp, synthetic construct
  misc_feature 1..34: note = primer #155 (IL2_N88V_F)
  source 1..34: mol_type = other DNA
cagggacttaatcagcgttatcaacgtatttgtt

SEQ ID NO: 369 - DNA, 34 bp, synthetic construct
  misc_feature 1..34: note = primer #156 (IL2_N88V_R)
  source 1..34: mol_type = other DNA
aacaaatacgttgataacgctgattaagtccctg

SEQ ID NO: 370 - DNA, 33 bp, synthetic construct
  misc_feature 1..33: note = primer #157 (IL2_I89F_F)
  source 1..33: mol_type = other DNA
gacttaatcagcaatttcaacgtaatagttctg

SEQ ID NO: 371 - DNA, 33 bp, synthetic construct
  misc_feature 1..33: note = primer #158 (IL2_I89F_R)
  source 1..33: mol_type = other DNA
cagaactattacgttgaaattgctgattaagtc

SEQ ID NO: 372 - DNA, 33 bp, synthetic construct
  misc_feature 1..33: note = primer #159 (IL2_V91E_I92F_F)
  source 1..33: mol_type = other DNA
agcaatatcaacgaattcgttctggaactaaag

SEQ ID NO: 373 - DNA, 33 bp, synthetic construct
  misc_feature 1..33: note = primer #160 (IL2_V91E_I92F_R)
  source 1..33: mol_type = other DNA
ctttagttccagaacgaattcgttgatattgct

SEQ ID NO: 374 - DNA, 33 bp, synthetic construct
  misc_feature 1..33: note = primer #161 (IL2_V91E_I92W_F)
  source 1..33: mol_type = other DNA
agcaatatcaacgaatgggttctggaactaaag

SEQ ID NO: 375 - DNA, 33 bp, synthetic construct
  misc_feature 1..33: note = primer #162 (IL2_V91E_I92W_R)
  source 1..33: mol_type = other DNA
ctttagttccagaacccattcgttgatattgct

SEQ ID NO: 376 - DNA, 34 bp, synthetic construct
  misc_feature 1..34: note = primer #163 (IL2_V91F_F)
  source 1..34: mol_type = other DNA
cagcaatatcaactttatagttctggaactaaag

SEQ ID NO: 377 - DNA, 34 bp, synthetic construct
  misc_feature 1..34: note = primer #164 (IL2_V91F_R)
  source 1..34: mol_type = other DNA
ctttagttccagaactataaagttgatattgctg

SEQ ID NO: 378 - DNA, 34 bp, synthetic construct
  misc_feature 1..34: note = primer #165 (IL2_V91T_F)
  source 1..34: mol_type = other DNA
cagcaatatcaacacaatagttctggaactaaag

SEQ ID NO: 379 - DNA, 34 bp, synthetic construct
  misc_feature 1..34: note = primer #166 (IL2_V91T_R)
  source 1..34: mol_type = other DNA
ctttagttccagaactattgtgttgatattgctg

SEQ ID NO: 380 - DNA, 32 bp, synthetic construct
  misc_feature 1..32: note = primer #167 (IL2_I92F_F)
  source 1..32: mol_type = other DNA
gcaatatcaacgtatttgttctggaactaaag

SEQ ID NO: 381 - DNA, 32 bp, synthetic construct
  misc_feature 1..32: note = primer #168 (IL2_I92F_R)
  source 1..32: mol_type = other DNA
ctttagttccagaacaaatacgttgatattgc

SEQ ID NO: 382 - DNA, 49 bp, synthetic construct
  misc_feature 1..49: note = primer #169 (IL2_I92F_F_long)
  source 1..49: mol_type = other DNA
gacttaatcagcaatatcaacgtatttgttctggaactaaagggatctg

SEQ ID NO: 383 - DNA, 49 bp, synthetic construct
  misc_feature 1..49: note = primer #170 (IL2_I92F_R_long)
  source 1..49: mol_type = other DNA
cagatccctttagttccagaacaaatacgttgatattgctgattaagtc

SEQ ID NO: 384 - DNA, 45 bp, synthetic construct
  misc_feature 1..45: note = primer #171 (IL2_I92F_F_long2)
  source 1..45: mol_type = other DNA
cttaatcagcaatatcaacgtatttgttctggaactaaagggatc

SEQ ID NO: 385 - DNA, 45 bp, synthetic construct
  misc_feature 1..45: note = primer #172 (IL2_I92F_R_long2)
  source 1..45: mol_type = other DNA
gatccctttagttccagaacaaatacgttgatattgctgattaag

SEQ ID NO: 386 - DNA, 32 bp, synthetic construct
  misc_feature 1..32: note = primer #173 (IL2_I92F_L94F_L96F_F)
  source 1..32: mol_type = other DNA
caacgtatttgttttcgaattcaagggatctg

SEQ ID NO: 387 - DNA, 32 bp, synthetic construct
  misc_feature 1..32: note = primer #174 (IL2_I92F_L94F_L96F_R)
  source 1..32: mol_type = other DNA
cagatcccttgaattcgaaaacaaatacgttg

SEQ ID NO: 388 - DNA, 39 bp, synthetic construct
  misc_feature 1..39: note = primer #175 (IL2_I92F_L94F_L96F_F)
  source 1..39: mol_type = other DNA
gcaatatcaacgtatttgttttcgaatttaagggatctg

SEQ ID NO: 389 - DNA, 39 bp, synthetic construct
  misc_feature 1..39: note = primer #176 (IL2_I92F_L94F_L96F_R)
  source 1..39: mol_type = other DNA
cagatcccttaaattcgaaaacaaatacgttgatattgc

SEQ ID NO: 390 - DNA, 39 bp, synthetic construct
  misc_feature 1..39: note = primer #177 (IL2_I92F_L94F_L96I_F)
  source 1..39: mol_type = other DNA
gcaatatcaacgtatttgttttcgaaattaagggatctg

SEQ ID NO: 391 - DNA, 39 bp, synthetic construct
  misc_feature 1..39: note = primer #178 (IL2_I92F_L94F_L96I_R)
  source 1..39: mol_type = other DNA
cagatcccttaatttcgaaaacaaatacgttgatattgc

SEQ ID NO: 392 - DNA, 39 bp, synthetic construct
  misc_feature 1..39: note = primer #179 (IL2_I92F_L94F_L96V_F)
  source 1..39: mol_type = other DNA
gcaatatcaacgtatttgttttcgaagtaaagggatctg

SEQ ID NO: 393 - DNA, 39 bp, synthetic construct
  misc_feature 1..39: note = primer #180 (IL2_I92F_L94F_L96V_R)
  source 1..39: mol_type = other DNA
cagatccctttacttcgaaaacaaatacgttgatattgc

SEQ ID NO: 394 - DNA, 33 bp, synthetic construct
  misc_feature 1..33: note = primer #181 (IL2_I92I_F)
  source 1..33: mol_type = other DNA
gcaatatcaacgtaattgttctggaactaaagg

SEQ ID NO: 395 - DNA, 33 bp, synthetic construct
  misc_feature 1..33: note = primer #182 (IL2_I92I_R)
  source 1..33: mol_type = other DNA
cctttagttccagaacaattacgttgatattgc

SEQ ID NO: 396 - DNA, 33 bp, synthetic construct
  misc_feature 1..33: note = primer #183 (IL2_I92L_F)
  source 1..33: mol_type = other DNA
gcaatatcaacgtattagttctggaactaaagg

SEQ ID NO: 397 - DNA, 33 bp, synthetic construct
  misc_feature 1..33: note = primer #184 (IL2_I92L_R)
  source 1..33: mol_type = other DNA
cctttagttccagaactaatacgttgatattgc

SEQ ID NO: 398 - DNA, 33 bp, synthetic construct
  misc_feature 1..33: note = primer #185 (IL2_I92W_F)
  source 1..33: mol_type = other DNA
agcaatatcaacgtatgggttctggaactaaag

SEQ ID NO: 399 - DNA, 33 bp, synthetic construct
  misc_feature 1..33: note = primer #186 (IL2_I92W_R)
  source 1..33: mol_type = other DNA
ctttagttccagaacccatacgttgatattgct

SEQ ID NO: 400 - DNA, 32 bp, synthetic construct
  misc_feature 1..32: note = primer #187 (IL2_I92Y_F)
  source 1..32: mol_type = other DNA
gcaatatcaacgtatatgttctggaactaaag

SEQ ID NO: 401 - DNA, 32 bp, synthetic construct
  misc_feature 1..32: note = primer #188 (IL2_I92Y_R)
  source 1..32: mol_type = other DNA
ctttagttccagaacatatacgttgatattgc

SEQ ID NO: 402 - DNA, 33 bp, synthetic construct
  misc_feature 1..33: note = primer #189 (IL2_L94F_L96F_F)
  source 1..33: mol_type = other DNA
cgtaatagttttcgaatttaagggatctgaaac

SEQ ID NO: 403 - DNA, 33 bp, synthetic construct
  misc_feature 1..33: note = primer #190 (IL2_L94F_L96F_R)
  source 1..33: mol_type = other DNA
gtttcagatcccttaaattcgaaaactattacg

SEQ ID NO: 404 - DNA, 33 bp, synthetic construct
  misc_feature 1..33: note = primer #191 (IL2_L94F_L96I_F)
  source 1..33: mol_type = other DNA
cgtaatagttttcgaaattaagggatctgaaac

SEQ ID NO: 405 - DNA, 33 bp, synthetic construct
  misc_feature 1..33: note = primer #192 (IL2_L94F_L96I_R)
  source 1..33: mol_type = other DNA
gtttcagatcccttaatttcgaaaactattacg

SEQ ID NO: 406 - DNA, 33 bp, synthetic construct
  misc_feature 1..33: note = primer #193 (IL2_L94F_L96V_F)
  source 1..33: mol_type = other DNA
cgtaatagttttcgaagtaaagggatctgaaac

SEQ ID NO: 407 - DNA, 33 bp, synthetic construct
  misc_feature 1..33: note = primer #194 (IL2_L94F_L96V_R)
  source 1..33: mol_type = other DNA
gtttcagatccctttacttcgaaaactattacg

SEQ ID NO: 408 - DNA, 30 bp, synthetic construct
  misc_feature 1..30: note = primer #195 (IL2_E95D_F)
  source 1..30: mol_type = other DNA
gttctggacctaaagggatctgaaacaaca

SEQ ID NO: 409 - DNA, 30 bp, synthetic construct
  misc_feature 1..30: note = primer #196 (IL2_E95D_R)
  source 1..30: mol_type = other DNA
tgttgtttcagatccctttaggtccagaac

SEQ ID NO: 410 - DNA, 33 bp, synthetic construct
  misc_feature 1..33: note = primer #197 (IL2_C125S_F)
  source 1..33: mol_type = other DNA
agatggattacctttagtcaaagcatcatctca

SEQ ID NO: 411 - DNA, 33 bp, synthetic construct
  misc_feature 1..33: note = primer #198 (IL2_C125S_R)
  source 1..33: mol_type = other DNA
tgagatgatgctttgactaaaggtaatccatct

SEQ ID NO: 412 - DNA, 34 bp, synthetic construct
  misc_feature 1..34: note = primer #199 (IL2_Q126T_F)
  source 1..34: mol_type = other DNA
gatggattacctttagtacaagcatcatctcaac

SEQ ID NO: 413 - DNA, 34 bp, synthetic construct
  misc_feature 1..34: note = primer #200 (IL2_Q126T_R)
  source 1..34: mol_type = other DNA
gttgagatgatgcttgtactaaaggtaatccatc

SEQ ID NO: 414 - DNA, 33 bp, synthetic construct
  misc_feature 1..33: note = primer #201 (IL2_desA1_F)
  source 1..33: mol_type = other DNA
taagaatatacatatgcctacttcaagttctac

SEQ ID NO: 415 - DNA, 33 bp, synthetic construct
  misc_feature 1..33: note = primer #202 (IL2_desA1_R)
  source 1..33: mol_type = other DNA
gtagaacttgaagtaggcatatgtatattctta

SEQ ID NO: 416 - DNA, 34 bp, synthetic construct
  misc_feature 1..34: note = primer #203 (IL2_NdeI_desA1_N-term)
  source 1..34: mol_type = other DNA
cgccatatgcctacttcaagttctacaaagaaaa

SEQ ID NO: 417 - DNA, 34 bp, synthetic construct
  misc_feature 1..34: note = primer #204 (IL2_BHI_C-term)
  source 1..34: mol_type = other DNA
cgggatcctcaagtcagtgttgagatgatgcttt

SEQ ID NO: 418 - protein, 12 aa, HOMO SAPIENS
ESKYGPPCPSCP

SEQ ID NO: 419 - protein, 11 aa, synthetic construct
  REGION 1..11: note = Variant of hinge region
ESKYGPPPSCP

SEQ ID NO: 420 - protein, 11 aa, synthetic construct
  REGION 1..11: note = Variant of hinge region
ESKYGPPCPSP

SEQ ID NO: 421 - protein, 10 aa, synthetic construct
  REGION 1..10: note = Variant of hinge region
ESKYGPPCPS

SEQ ID NO: 422 - protein, 10 aa, synthetic construct
  REGION 1..10: note = Variant of hinge region
ESKYGPPCPP

SEQ ID NO: 423 - protein, 8 aa, synthetic construct
  REGION 1..8: note = Variant of hinge region
KYGPPCPS

SEQ ID NO: 424 - protein, 8 aa, synthetic construct
  REGION 1..8: note = Variant of hinge region
ESKYGPPC

SEQ ID NO: 425 - protein, 7 aa, synthetic construct
  REGION 1..7: note = Variant of hinge region
EKYGPPC

SEQ ID NO: 426 - protein, 6 aa, synthetic construct
  REGION 1..6: note = Variant of hinge region
ESPSCP

SEQ ID NO: 427 - protein, 5 aa, synthetic construct
  REGION 1..5: note = Variant of hinge region
EPSCP

SEQ ID NO: 428 - protein, 4 aa, synthetic construct
  REGION 1..4: note = Variant of hinge region
PSCP

SEQ ID NO: 429 - protein, 10 aa, synthetic construct
  REGION 1..10: note = Variant of hinge region
ESKYGPPSCP

SEQ ID NO: 430 - protein, 9 aa, synthetic construct
  REGION 1..9: note = Variant of hinge region
KYGPPPSCP

SEQ ID NO: 431 - protein, 9 aa, synthetic construct
  REGION 1..9: note = Variant of hinge region
ESKYGPSCP

SEQ ID NO: 432 - protein, 8 aa, synthetic construct
  REGION 1..8: note = Variant of hinge region
ESKYGPPC

SEQ ID NO: 433 - protein, 7 aa, synthetic construct
  REGION 1..7: note = Variant of hinge region
KYGPPCP

SEQ ID NO: 434 - protein, 7 aa, synthetic construct
  REGION 1..7: note = Variant of hinge region
ESKPSCP

SEQ ID NO: 435 - protein, 6 aa, synthetic construct
  REGION 1..6: note = Variant of hinge region
ESPSCP

SEQ ID NO: 436 - protein, 4 aa, synthetic construct
  REGION 1..4: note = Variant of hinge region
EPSC

SEQ ID NO: 437 - skipped

SEQ ID NO: 438 - protein, 221 aa, homo sapiens
PSCPAPEFLGGPSVFLFPPKPKDTLMISRTPEVTCVVVDVSQEDPEVQFNWYVDGVEVHNAKTKPREEQFNSTYRVVSVLTVLHQDWLNGKEYKCKVSNKGLPSSIEKTISKAKGQPREPQVYTLPPSQEEMTKNQVSLTCLVKGFYPSDIAVEWESNGQPENNYKTTPPVLDSDGSFFLYSRLTVDKSRWQEGNVFSCSVMHEALHNHYTQKSLSLSLGK

SEQ ID NO: 439 - protein, 442 aa, Homo sapiens
  REGION 1..442: note = MISC_FEATURE - Amino acids at position 1 to 442 form Human Immunoglobulin G4 Fc Fragment (homodimer)
  REGION 1..221: note = MISC_FEATURE - Amino acids at position 1 to 221 form one monomer
  REGION 222..442: note = MISC_FEATURE - Amino acids at position 222 to 442 form one monomer
  DISULFID 3..224: note = Amino acids at position 3 and position 224 form an inter-disulfide bond
  DISULFID 35..95: note = Amino acids at position 35 and position 95 form an intra-chain disulfide bond
  DISULFID 141..199: note = Amino acids at position 141 and position 199 form an intra-chain disulfide bond
  DISULFID 256..316: note = Amino acids at position 256 and position 316 form an intra-chain disulfide bond
  DISULFID 362..420: note = Amino acids at position 362 and position 420 form an intra-chain disulfide bond
PSCPAPEFLGGPSVFLFPPKPKDTLMISRTPEVTCVVVDVSQEDPEVQFNWYVDGVEVHNAKTKPREEQFNSTYRVVSVLTVLHQDWLNGKEYKCKVSNKGLPSSIEKTISKAKGQPREPQVYTLPPSQEEMTKNQVSLTCLVKGFYPSDIAVEWESNGQPENNYKTTPPVLDSDGSFFLYSRLTVDKSRWQEGNVFSCSVMHEALHNHYTQKSLSLSLGKPSCPAPEFLGGPSVFLFPPKPKDTLMISRTPEVTCVVVDVSQEDPEVQFNWYVDGVEVHNAKTKPREEQFNSTYRVVSVLTVLHQDWLNGKEYKCKVSNKGLPSSIEKTISKAKGQPREPQVYTLPPSQEEMTKNQVSLTCLVKGFYPSDIAVEWESNGQPENNYKTTPPVLDSDGSFFLYSRLTVDKSRWQEGNVFSCSVMHEALHNHYTQKSLSLSLGK